European Patent Specification EP 3 130 607 B1, published April 17, 2024. Title: MUC1 ANTIBODY. Applicant: Minerva Biochtechnologies Corporation BAMDAD, Cynthia. The sequence listing filed with the application follows.

SEQUENCE LISTING (374 sequences)

SEQ ID NO: 1 - protein, 45 aa, Artificial Sequence
  membrane proximal extracellular region of MUC1 from amino acid 1110 to 1155
GTINVHDVETQFNQYKTEAASRYNLTISDVSVSDVPFPFSAQSGA

SEQ ID NO: 2 - protein, 45 aa, Artificial Sequence
  variant of membrane proximal extracellular region of MUC1 from amino acid 1110 to 1155
GTINVHDVETQFNQYKTEAASPYNLTISDVSVSDVPFPFSAQSGA

SEQ ID NO: 3 - DNA, 36 bp, Artificial Sequence
  HindIII restriction site
ggaaagcttatagacagatgggggtgtcgttttggc

SEQ ID NO: 4 - DNA, 32 bp, Artificial Sequence
  HindIII restriction site
ggaaagcttcttgaccaggcatcctagagtca

SEQ ID NO: 5 - DNA, 33 bp, Artificial Sequence
  HindIII restriction site
ggaaagcttaggggccagtggatagactgatgg

SEQ ID NO: 6 - DNA, 32 bp, Artificial Sequence
  EcoRI restriction site
  misc_feature (18)..(18): n is a, c, g, or t
cttccggaattcsargtnmagctgsagsagtc

SEQ ID NO: 7 - DNA, 35 bp, Artificial Sequence
  EcoRI restriction site
  misc_feature (18)..(18): n is a, c, g, or t
cttccggaattcsargtnmagctgsagsagtcwgg

SEQ ID NO: 8 - DNA, 30 bp, Artificial Sequence
  SalI restriction site
ggtgtcgacggatacagttggtgcagcatc

SEQ ID NO: 9 - DNA, 32 bp, Artificial Sequence
  SacI restriction site
gggagctcgayattgtgmtsacmcarwctmca

SEQ ID NO: 10 - DNA, 390 bp, Artificial Sequence
  MIN-C2 Heavy chain variable region
gaggtccagctggaggagtcagggggaggcttagtgaagcctggagggtccctgaaactctcctgtgcagcctctggattcactttcagtggctatgccatgtcttgggttcgccagactccggagaagaggctggagtgggtcgcaaccattagtagtggtggtacttatatctactatccagacagtgtgaaggggcgattcaccatctccagagacaatgccaagaacaccctgtacctgcaaatgagcagtctgaggtctgaggacacggccatgtattactgtgcaagacttgggggggataattactacgaatacttcgatgtctggggcgcagggaccacggtcaccgtctcctccgccaaaacgacacccccatctgtctat

SEQ ID NO: 11 - protein, 130 aa, Artificial Sequence
  MIN-C2 Heavy chain variable region
EVQLEESGGGLVKPGGSLKLSCAASGFTFSGYAMSWVRQTPEKRLEWVATISSGGTYIYYPDSVKGRFTISRDNAKNTLYLQMSSLRSEDTAMYYCARLGGDNYYEYFDVWGAGTTVTVSSAKTTPPSVY

SEQ ID NO: 12 - DNA, 360 bp, Artificial Sequence
  MIN-C2 Kappa chain variable region
gacattgtgatcacacagtctacagcttccttaggtgtatctctggggcagagggccaccatctcatgcagggccagcaaaagtgtcagtacatctggctatagttatatgcactggtaccaacagagaccaggacagccacccaaactcctcatctatcttgcatccaacctagaatctggggtccctgccaggttcagtggcagtgggtctgggacagacttcaccctcaacatccatcctgtggaggaggaggatgctgcaacctattactgtcagcacagtagggagcttccgttcacgttcggaggggggaccaagctggagataaaacgggctgatgctgcaccaactgtatcc

SEQ ID NO: 13 - protein, 120 aa, Artificial Sequence
  MIN-C2 Kappa chain variable region
DIVITQSTASLGVSLGQRATISCRASKSVSTSGYSYMHWYQQRPGQPPKLLIYLASNLESGVPARFSGSGSGTDFTLNIHPVEEEDAATYYCQHSRELPFTFGGGTKLEIKRADAAPTVS

SEQ ID NO: 14 - DNA, 45 bp, Artificial Sequence
  Linker
ggtggaggcggatcaggtggaggcggatcaggtggaggcggatca

SEQ ID NO: 15 - DNA, 795 bp, Artificial Sequence
  MIN-C2 Heavy chain-linker-light chain
gaggtccagctggaggagtcagggggaggcttagtgaagcctggagggtccctgaaactctcctgtgcagcctctggattcactttcagtggctatgccatgtcttgggttcgccagactccggagaagaggctggagtgggtcgcaaccattagtagtggtggtacttatatctactatccagacagtgtgaaggggcgattcaccatctccagagacaatgccaagaacaccctgtacctgcaaatgagcagtctgaggtctgaggacacggccatgtattactgtgcaagacttgggggggataattactacgaatacttcgatgtctggggcgcagggaccacggtcaccgtctcctccgccaaaacgacacccccatctgtctatggtggaggcggatcaggtggaggcggatcaggtggaggcggatcagacattgtgatcacacagtctacagcttccttaggtgtatctctggggcagagggccaccatctcatgcagggccagcaaaagtgtcagtacatctggctatagttatatgcactggtaccaacagagaccaggacagccacccaaactcctcatctatcttgcatccaacctagaatctggggtccctgccaggttcagtggcagtgggtctgggacagacttcaccctcaacatccatcctgtggaggaggaggatgctgcaacctattactgtcagcacagtagggagcttccgttcacgttcggaggggggaccaagctggagataaaacgggctgatgctgcaccaactgtatcc

SEQ ID NO: 16 - DNA, 798 bp, Artificial Sequence
  MIN-C2 Heavy chain-linker-light chain-Cys
gaggtccagctggaggagtcagggggaggcttagtgaagcctggagggtccctgaaactctcctgtgcagcctctggattcactttcagtggctatgccatgtcttgggttcgccagactccggagaagaggctggagtgggtcgcaaccattagtagtggtggtacttatatctactatccagacagtgtgaaggggcgattcaccatctccagagacaatgccaagaacaccctgtacctgcaaatgagcagtctgaggtctgaggacacggccatgtattactgtgcaagacttgggggggataattactacgaatacttcgatgtctggggcgcagggaccacggtcaccgtctcctccgccaaaacgacacccccatctgtctatggtggaggcggatcaggtggaggcggatcaggtggaggcggatcagacattgtgatcacacagtctacagcttccttaggtgtatctctggggcagagggccaccatctcatgcagggccagcaaaagtgtcagtacatctggctatagttatatgcactggtaccaacagagaccaggacagccacccaaactcctcatctatcttgcatccaacctagaatctggggtccctgccaggttcagtggcagtgggtctgggacagacttcaccctcaacatccatcctgtggaggaggaggatgctgcaacctattactgtcagcacagtagggagcttccgttcacgttcggaggggggaccaagctggagataaaacgggctgatgctgcaccaactgtatcctgt

SEQ ID NO: 17 - protein, 267 aa, Artificial Sequence
  MIN-C2 Heavy chain-linker-light chain
EVQLEESGGGLVKPGGSLKLSCAASGFTFSGYAMSWVRQTPEKRLEWVATISSGGTYIYYPDSVKGRFTISRDNAKNTLYLQMSSLRSEDTAMYYCARLGGDNYYEYFDVWGAGTTVTVSSAKTTPPSVYGGGGSGGGGSGGGGSDIVITQSTASLGVSLGQRATISCRASKSVSTSGYSYMHWYQQRPGQPPKLLIYLASNLESGVPARFSGSGSGTDFTLNIHPVEEEDAATYYCQHSRELPFTFGGGTKLEIKRADAAPTVSVD

SEQ ID NO: 18 - protein, 266 aa, Artificial Sequence
  MIN-C2 Heavy chain-linker-light chain-Cys
EVQLEESGGGLVKPGGSLKLSCAASGFTFSGYAMSWVRQTPEKRLEWVATISSGGTYIYYPDSVKGRFTISRDNAKNTLYLQMSSLRSEDTAMYYCARLGGDNYYEYFDVWGAGTTVTVSSAKTTPPSVYGGGGSGGGGSGGGGSDIVITQSTASLGVSLGQRATISCRASKSVSTSGYSYMHWYQQRPGQPPKLLIYLASNLESGVPARFSGSGSGTDFTLNIHPVEEEDAATYYCQHSRELPFTFGGGTKLEIKRADAAPTVSC

SEQ ID NO: 19 - DNA, 393 bp, Artificial Sequence
  MIN-E6 Heavy chain-7 variable region
gaggttaagctggaggagtctgggggagacttagtgaagcctggagggtccctgaaactctcctgtgcagcctctggattcactttcagtagatatggcatgtcttgggttcgccagactccagacaagaggctggagtgggtcgcaaccattagtagtggtggtacttacatctactatccagacagtgtgaaggggcgattcaccatctccagagacaatgccaagaacaccctgtacctgcaaatgagcagtctgaagtctgaggacacagccatgtattactgtgcaagggataactacggtagtagctacgactatgctatggactactggggtcaaggaacctcagtcaccgtctcctcagccaaaacaacagccccatcggtctat

SEQ ID NO: 20 - protein, 131 aa, Artificial Sequence
  MIN-E6 Heavy chain-7 variable region
EVKLEESGGDLVKPGGSLKLSCAASGFTFSRYGMSWVRQTPDKRLEWVATISSGGTYIYYPDSVKGRFTISRDNAKNTLYLQMSSLKSEDTAMYYCARDNYGSSYDYAMDYWGQGTSVTVSSAKTTAPSVY

SEQ ID NO: 21 - DNA, 456 bp, Artificial Sequence
  MIN-E6 Heavy chain-8 variable region
gaggtaaagctggaggagtctgggggagacttagtgaagcctggagggtccctgaaactctcctgtgtagtctctggattcactttcagtagatatggcatgtcttgggttcgccagactccaggcaagaggctggagtgggtcgcaaccattagtggtggcggtacttacatctactatccagacagtgtgaaggggcgattcaccatctccagagacaatgccaagaacaccctgtacctgcaaatgagcagtctgaagtctgaggacacagccatgtatcactgtacaagggataactacggtaggaactacgactacggtatggactactggggtcaaggaacctcagtcaccgtctcctcagccaaaacaacagccccatcggtctatccactggcccctgtgtgtggagatacaactggctcctcggtgactctaggatgcctggtcaag

SEQ ID NO: 22 - protein, 152 aa, Artificial Sequence
  MIN-E6 Heavy chain-8 variable region
EVKLEESGGDLVKPGGSLKLSCVVSGFTFSRYGMSWVRQTPGKRLEWVATISGGGTYIYYPDSVKGRFTISRDNAKNTLYLQMSSLKSEDTAMYHCTRDNYGRNYDYGMDYWGQGTSVTVSSAKTTAPSVYPLAPVCGDTTGSSVTLGCLVK

SEQ ID NO: 23 - DNA, 345 bp, Artificial Sequence
  MIN-E6 Kappa chain variable region
gatattgtgatcacccagactacagcaatcatgtctgcatctccaggggaggaggtcaccctaacctgcagtgccacctcaagtgtaagttacatacactggttccagcagaggccaggcacttctcccaaactctggatttatagcacatccaacctggcttctggagtccctgttcgcttcagtggcagtggatatgggacctcttactctctcacaatcagccgaatggaggctgaagatgctgccacttattactgccagcaaaggagtagttccccattcacgttcggctcggggacaaagttggaaataaaacgggctgatgctgcaccaactgtatcc

SEQ ID NO: 24 - protein, 115 aa, Artificial Sequence
  MIN-E6 Kappa chain variable region
DIVITQTTAIMSASPGEEVTLTCSATSSVSYIHWFQQRPGTSPKLWIYSTSNLASGVPVRFSGSGYGTSYSLTISRMEAEDAATYYCQQRSSSPFTFGSGTKLEIKRADAAPTVS

SEQ ID NO: 25 - DNA, 846 bp, Artificial Sequence
  MIN-E6 scFv: Heavy chain 7-linker-light chain (VH + linker + VL)
gaggttaagctggaggagtctgggggagacttagtgaagcctggagggtccctgaaactctcctgtgcagcctctggattcactttcagtagatatggcatgtcttgggttcgccagactccagacaagaggctggagtgggtcgcaaccattagtagtggtggtacttacatctactatccagacagtgtgaaggggcgattcaccatctccagagacaatgccaagaacaccctgtacctgcaaatgagcagtctgaagtctgaggacacagccatgtattactgtgcaagggataactacggtagtagctacgactatgctatggactactggggtcaaggaacctcagtcaccgtctcctcagccaaaacaacagccccatcggtctatccactggcccctgtgtgtggagatacaactggctcctcggtgactctaggatgcctggtcaagggtggaggcggatcaggtggaggcggatcaggtggaggcggatcagatattgtgatcacccagactacagcaatcatgtctgcatctccaggggaggaggtcaccctaacctgcagtgccacctcaagtgtaagttacatacactggttccagcagaggccaggcacttctcccaaactctggatttatagcacatccaacctggcttctggagtccctgttcgcttcagtggcagtggatatgggacctcttactctctcacaatcagccgaatggaggctgaagatgctgccacttattactgccagcaaaggagtagttccccattcacgttcggctcggggacaaagttggaaataaaacgggctgatgctgcaccaactgtatcc

SEQ ID NO: 26 - DNA, 849 bp, Artificial Sequence
  MIN-E6 scFv - Cys: Heavy chain 7-linker-light chain-Cys (VH + linker + VL + Cys)
gaggttaagctggaggagtctgggggagacttagtgaagcctggagggtccctgaaactctcctgtgcagcctctggattcactttcagtagatatggcatgtcttgggttcgccagactccagacaagaggctggagtgggtcgcaaccattagtagtggtggtacttacatctactatccagacagtgtgaaggggcgattcaccatctccagagacaatgccaagaacaccctgtacctgcaaatgagcagtctgaagtctgaggacacagccatgtattactgtgcaagggataactacggtagtagctacgactatgctatggactactggggtcaaggaacctcagtcaccgtctcctcagccaaaacaacagccccatcggtctatccactggcccctgtgtgtggagatacaactggctcctcggtgactctaggatgcctggtcaagggtggaggcggatcaggtggaggcggatcaggtggaggcggatcagatattgtgatcacccagactacagcaatcatgtctgcatctccaggggaggaggtcaccctaacctgcagtgccacctcaagtgtaagttacatacactggttccagcagaggccaggcacttctcccaaactctggatttatagcacatccaacctggcttctggagtccctgttcgcttcagtggcagtggatatgggacctcttactctctcacaatcagccgaatggaggctgaagatgctgccacttattactgccagcaaaggagtagttccccattcacgttcggctcggggacaaagttggaaataaaacgggctgatgctgcaccaactgtatcctgt

SEQ ID NO: 27 - protein, 282 aa, Artificial Sequence
  MIN-E6 scFv Heavy chain 7-linker-light chain (VH + linker + VL)
EVKLEESGGDLVKPGGSLKLSCAASGFTFSRYGMSWVRQTPDKRLEWVATISSGGTYIYYPDSVKGRFTISRDNAKNTLYLQMSSLKSEDTAMYYCARDNYGSSYDYAMDYWGQGTSVTVSSAKTTAPSVYPLAPVCGDTTGSSVTLGCLVKGGGGSGGGGSGGGGSDIVITQTTAIMSASPGEEVTLTCSATSSVSYIHWFQQRPGTSPKLWIYSTSNLASGVPVRFSGSGYGTSYSLTISRMEAEDAATYYCQQRSSSPFTFGSGTKLEIKRADAAPTVS

SEQ ID NO: 28 - protein, 283 aa, Artificial Sequence
  MIN-E6 scFv-Cys Heavy chain 7-linker-light chain-Cys (VH + linker + VL + Cys)
EVKLEESGGDLVKPGGSLKLSCAASGFTFSRYGMSWVRQTPDKRLEWVATISSGGTYIYYPDSVKGRFTISRDNAKNTLYLQMSSLKSEDTAMYYCARDNYGSSYDYAMDYWGQGTSVTVSSAKTTAPSVYPLAPVCGDTTGSSVTLGCLVKGGGGSGGGGSGGGGSDIVITQTTAIMSASPGEEVTLTCSATSSVSYIHWFQQRPGTSPKLWIYSTSNLASGVPVRFSGSGYGTSYSLTISRMEAEDAATYYCQQRSSSPFTFGSGTKLEIKRADAAPTVSC

SEQ ID NO: 29 - DNA, 846 bp, Artificial Sequence
  MIN-E6 Heavy chain 8-linker-light chain
gaggtaaagctggaggagtctgggggagacttagtgaagcctggagggtccctgaaactctcctgtgtagtctctggattcactttcagtagatatggcatgtcttgggttcgccagactccaggcaagaggctggagtgggtcgcaaccattagtggtggcggtacttacatctactatccagacagtgtgaaggggcgattcaccatctccagagacaatgccaagaacaccctgtacctgcaaatgagcagtctgaagtctgaggacacagccatgtatcactgtacaagggataactacggtaggaactacgactacggtatggactactggggtcaaggaacctcagtcaccgtctcctcagccaaaacaacagccccatcggtctatccactggcccctgtgtgtggagatacaactggctcctcggtgactctaggatgcctggtcaagggtggaggcggatcaggtggaggcggatcaggtggaggcggatcagatattgtgatcacccagactacagcaatcatgtctgcatctccaggggaggaggtcaccctaacctgcagtgccacctcaagtgtaagttacatacactggttccagcagaggccaggcacttctcccaaactctggatttatagcacatccaacctggcttctggagtccctgttcgcttcagtggcagtggatatgggacctcttactctctcacaatcagccgaatggaggctgaagatgctgccacttattactgccagcaaaggagtagttccccattcacgttcggctcggggacaaagttggaaataaaacgggctgatgctgcaccaactgtatcc

SEQ ID NO: 30 - DNA, 849 bp, Artificial Sequence
  MIN-E6 Heavy chain 8-linker-light chain-Cys
gaggtaaagctggaggagtctgggggagacttagtgaagcctggagggtccctgaaactctcctgtgtagtctctggattcactttcagtagatatggcatgtcttgggttcgccagactccaggcaagaggctggagtgggtcgcaaccattagtggtggcggtacttacatctactatccagacagtgtgaaggggcgattcaccatctccagagacaatgccaagaacaccctgtacctgcaaatgagcagtctgaagtctgaggacacagccatgtatcactgtacaagggataactacggtaggaactacgactacggtatggactactggggtcaaggaacctcagtcaccgtctcctcagccaaaacaacagccccatcggtctatccactggcccctgtgtgtggagatacaactggctcctcggtgactctaggatgcctggtcaagggtggaggcggatcaggtggaggcggatcaggtggaggcggatcagatattgtgatcacccagactacagcaatcatgtctgcatctccaggggaggaggtcaccctaacctgcagtgccacctcaagtgtaagttacatacactggttccagcagaggccaggcacttctcccaaactctggatttatagcacatccaacctggcttctggagtccctgttcgcttcagtggcagtggatatgggacctcttactctctcacaatcagccgaatggaggctgaagatgctgccacttattactgccagcaaaggagtagttccccattcacgttcggctcggggacaaagttggaaataaaacgggctgatgctgcaccaactgtatcctgt

SEQ ID NO: 31 - protein, 282 aa, Artificial Sequence
  MIN-E6 Heavy chain 8-linker-light chain
EVKLEESGGDLVKPGGSLKLSCVVSGFTFSRYGMSWVRQTPGKRLEWVATISGGGTYIYYPDSVKGRFTISRDNAKNTLYLQMSSLKSEDTAMYHCTRDNYGRNYDYGMDYWGQGTSVTVSSAKTTAPSVYPLAPVCGDTTGSSVTLGCLVKGGGGSGGGGSGGGGSDIVITQTTAIMSASPGEEVTLTCSATSSVSYIHWFQQRPGTSPKLWIYSTSNLASGVPVRFSGSGYGTSYSLTISRMEAEDAATYYCQQRSSSPFTFGSGTKLEIKRADAAPTVS

SEQ ID NO: 32 - protein, 283 aa, Artificial Sequence
  MIN-E6 Heavy chain 8-linker-light chain-Cys
EVKLEESGGDLVKPGGSLKLSCVVSGFTFSRYGMSWVRQTPGKRLEWVATISGGGTYIYYPDSVKGRFTISRDNAKNTLYLQMSSLKSEDTAMYHCTRDNYGRNYDYGMDYWGQGTSVTVSSAKTTAPSVYPLAPVCGDTTGSSVTLGCLVKGGGGSGGGGSGGGGSDIVITQTTAIMSASPGEEVTLTCSATSSVSYIHWFQQRPGTSPKLWIYSTSNLASGVPVRFSGSGYGTSYSLTISRMEAEDAATYYCQQRSSSPFTFGSGTKLEIKRADAAPTVSC

SEQ ID NO: 33 - DNA, 38 bp, Artificial Sequence
  EcoRI restriction site
gggaattccaccatggratgsagctgkgtmatsctctt

SEQ ID NO: 34 - DNA, 38 bp, Artificial Sequence
  EcoRI restriction site
gggaattccaccatgracttcgggytgagctkggtttt

SEQ ID NO: 35 - DNA, 37 bp, Artificial Sequence
  EcoRI restriction site
gggaattccaccatggctgtcttggggctgctcttct

SEQ ID NO: 36 - DNA, 30 bp, Artificial Sequence
  EcoRI restriction site
gggaattccaccatggrcagrcttacwtyy

SEQ ID NO: 37 - DNA, 31 bp, Artificial Sequence
  XhoI restriction site
ctacctcgagckyggtsytgctggcygggtg

SEQ ID NO: 38 - DNA, 38 bp, Artificial Sequence
  EcoRI restriction site
gggaattccaccatggattttcaggtgcagattttcag

SEQ ID NO: 39 - DNA, 38 bp, Artificial Sequence; identical to SEQ ID NO: 38
  EcoRI restriction site

SEQ ID NO: 40 - DNA, 39 bp, Artificial Sequence
  EcoRI restriction site
gggaattccaccatgragtcacakacycaggtcttyrta

SEQ ID NO: 41 - DNA, 39 bp, Artificial Sequence
  EcoRI restriction site
gggaattccaccatgaggkccccwgctcagytyctkggr

SEQ ID NO: 42 - DNA, 36 bp, Artificial Sequence
  EcoRI restriction site
gggaattccaccatgaagttgcctgttaggctgttg

SEQ ID NO: 43 - DNA, 34 bp, Artificial Sequence
  EcoRI restriction site
gggaattccaccatgatgagtcctgcccagttcc

SEQ ID NO: 44 - DNA, 33 bp, Artificial Sequence
  XhoI restriction site
ctacctcgagttaacactcattcctgttgaagc

SEQ ID NO: 45 - DNA, 639 bp, Artificial Sequence
  MIN-C2 Fab Heavy chain
gaggtccagctggaggagtctgggggaggcttagtgaagcctggagggtccctgaaactctcctgtgcagcctctggattcactttcagtggctatgccatgtcttgggttcgccagactccggagaagaggctggagtgggtcgcaaccattagtagtggtggtacttatatctactatccagacagtgtgaaggggcgattcaccatctccagagacaatgccaagaacaccctgtacctgcaaatgagcagtctgaggtctgaggacacggccatgtattactgtgcaagacttgggggggataattactacgaatacttcgatgtctggggcgcagggaccacggtcaccgtctcctccgccaaaacgacacccccatctgtctatccactggcccctggatctgctgcccaaactaactccatggtgaccctgggatgcctggtcaagggctatttccctgagccagtgacagtgacctggaactctggatccctgtccagcggtgtgcacaccttcccagctgtcctgcagtctgacctctacactctgagcagctcagtgactgtcccctccagcacctggcccagcgagaccgtcacctgcaacgttgcccacccagccagcaggaccgcg

SEQ ID NO: 46 - DNA, 654 bp, Artificial Sequence
  MIN-C2 Fab Kappa chain
gacattgtgatcacacagtctacagcttccttaggtgtatctctggggcagagggccaccatctcatgcagggccagcaaaagtgtcagtacatctggctatagttatatgcactggtaccaacagagaccaggacagccacccaaactcctcatctatcttgcatccaacctagaatctggggtccctgccaggttcagtggcagtgggtctgggacagacttcaccctcaacatccatcctgtggaggaggaggatgctgcaacctattactgtcagcacagtagggagcttccgttcacgttcggaggggggaccaagctggagataaaacgggctgatgctgcaccaactgtatccatcttcccaccatccagtgagcagttaacatctggaggtgcctcagtcgtgtgcttcttgaacaacttctaccccaaagacatcaatgtcaagtggaagattgatggcagtgaacgacaaaatggcgtcctgaacagttggactgatcaggacagcaaagacagcacctacagcatgagcagcaccctcacgttgaccaaggacgagtatgaacgacataacagctatacctgtgaggccactcacaagacatcaacttcacccattgtcaagagcttcaacaggaatgagtgt

SEQ ID NO: 47 - protein, 213 aa, Artificial Sequence
  MIN-C2 Fab Heavy chain
EVQLEESGGGLVKPGGSLKLSCAASGFTFSGYAMSWVRQTPEKRLEWVATISSGGTYIYYPDSVKGRFTISRDNAKNTLYLQMSSLRSEDTAMYYCARLGGDNYYEYFDVWGAGTTVTVSSAKTTPPSVYPLAPGSAAQTNSMVTLGCLVKGYFPEPVTVTWNSGSLSSGVHTFPAVLQSDLYTLSSSVTVPSSTWPSETVTCNVAHPASRTA

SEQ ID NO: 48 - protein, 218 aa, Artificial Sequence
  MIN-C2 Fab Kappa chain
DIVITQSTASLGVSLGQRATISCRASKSVSTSGYSYMHWYQQRPGQPPKLLIYLASNLESGVPARFSGSGSGTDFTLNIHPVEEEDAATYYCQHSRELPFTFGGGTKLEIKRADAAPTVSIFPPSSEQLTSGGASVVCFLNNFYPKDINVKWKIDGSERQNGVLNSWTDQDSKDSTYSMSSTLTLTKDEYERHNSYTCEATHKTSTSPIVKSFNRNEC

SEQ ID NO: 49 - protein, 107 aa, Artificial Sequence
  MIN-C2 light CL region amino acid sequence
RADAAPTVSIFPPSSEQLTSGGASVVCFLNNFYPKDINVKWKIDGSERQNGVLNSWTDQDSKDSTYSMSSTLTLTKDEYERHNSYTCEATHKTSTSPIVKSFNRNEC

SEQ ID NO: 50 - protein, 106 aa, Artificial Sequence
  MIN-C2 heavy chain CH1 region amino acid sequence
FDVWGAGTTVTVSSAKTTPPSVYPLAPGSAAQTNSMVTLGCLVKGYFPEPVTVTWNSGSLSSGVHTFPAVLQSDLYTLSSSVTVPSSTWPSETVTCNVAHPASRTA

SEQ ID NO: 51 - protein, 115 aa, Artificial Sequence
  MIN- A2-1 light chain variable region amino acid sequence
DIVLTQSTEIMSASPGEKVTITCSASSSISYIHWFQQKPGTSPKLWIFGTSNLASGVPARFSGSGSGTSYSLTVSRMEAEDTATYYCQQRSNYPFTFGSGTKLQIKRADAAPTVS

SEQ ID NO: 52 - protein, 115 aa, Artificial Sequence
  MIN-A2-2 light chain variable region amino acid sequence
DIVMTQSPAIMSASPGEKVTMTCSASSSVSYMHWFQQKPGTSPKLWIYSTSNLASGAPARFSGSGSGTSYSLTVSRMESEDAATYYCQQRSSYPSTFGGGTKLEIKRADAAPTVS

SEQ ID NO: 53 - protein, 115 aa, Artificial Sequence
  MIN-C9-1 light chain variable region amino acid sequence
DIVLTQTTAIMSASPGEKVTITCSASSSVSYMYWFQQKPGTSPKLWIYSTSNLASGVPARFSGSGSGTSYSLTISRMEAEDAATYYCQQRSSYPSTFGGGTKLEIKRADAAPTVS

SEQ ID NO: 54 - protein, 115 aa, Artificial Sequence
  MIN-C9-2 light chain variable region amino acid sequence
DIVITQSTAIMSASPGEKVTITCSASSSVSYTYWFQQKPGTSPKLWIYSTSNLASGVPARFSGSGSGTSYSLTISRMEAEDAATYYCQQRSSYPSTFGGGTKLEIKRADAAPTVS

SEQ ID NO: 55 - protein, 115 aa, Artificial Sequence
  MIN-D7-1 light chain variable region amino acid sequence
DIVITQTPAIMSASPGEKVTMTCSASSSVSYMHWFQQKPGTSPKLWIYSTSNLASGVPARFSGSGSGTSYSLTVSRMESEDAATYYCQQRSSYPSTFGGGTKLEIKRADAAPTVS

SEQ ID NO: 56 - protein, 115 aa, Artificial Sequence
  MIN-D7-2 light chain variable region amino acid sequence
DIVLTQSTAIMSASPGEKVTMTCSASSSVSYMHWFQQKPGTSPKLWIYSTSNLASGVPARFSGSGSGTSYSLTVSRMESEDAATYYCQQRSSYPSTFGGGTKLEIKRADAAPTVS

SEQ ID NO: 57 - protein, 115 aa, Artificial Sequence
  MIN-F2-1 light chain variable region amino acid sequence
DIVMTQSPEIMSASPGEKVTITCSASSSISYIHWFQQKPGTSPKLWIFGTSNLASGVPARFSGSGSGTSYSLTVSRMEAEDTATYYCQQRSNYPFTFGSGTKLQIKRADAAPTVS

SEQ ID NO: 58 - protein, 115 aa, Artificial Sequence
  MIN-F2-2 light chain variable region amino acid sequence
DIVITQSTEIMSASPGEKVTITCSASSSISYIHWFQQKPGTSPKLWIFGTSNLASGVPARFSGSGSGTSYSLTVSRMEAEDTATYYCQQRSNYPFTFGSGTKLQIKRADAAPTVS

SEQ ID NO: 59 - protein, 130 aa, Artificial Sequence
  MIN-A2-1 heavy chain variable region amino acid sequence
EVKLQESGPELKKPGETVEISCKASGYTFTNYGMNWVKQAPGKGLKWMGWINTYTGEPTYAGDFKGRFAFSLETSASTAYLQINTLKNEDTATYFCARSGDGYWYYAMDYWGQGTSVTVSSAKTTPPSVY

SEQ ID NO: 60 - protein, 130 aa, Artificial Sequence
  MIN-A2-2 heavy chain variable region amino acid sequence
EVQLQQSGPELKKPGETVKISCKASGYTFTNYGMNWVKQAPGKGLKWMGWINTYTGEPTYAGDFKGRFAFSLETSASTAYLQINTLKNEDTATYFCARSGDGYWYYAMDYWGQGTSVTVSSAKTTPPSVY

SEQ ID NO: 61 - protein, 130 aa, Artificial Sequence
  MIN-C9-1 heavy chain variable region amino acid sequence
QVQLQESGPELKQPGETVKISCKASGYTFTNNGMNWVKQAPGKGLKWMGWINTYTGEPTYADDFKGRFAFSLDTSASTAYLQINNLKNEDMATYFCARTGTARAFYAMDYWGQGTSVTVSSTKTTAPSVY

SEQ ID NO: 62 - protein, 130 aa, Artificial Sequence
  MIN-C9-2 heavy chain variable region amino acid sequence
QVQLQQSGPELKQPGETVKISCKASGYTFTNNGMNWVKQAPGKGLKWMGWINTYTGEPTYADDFKGRFAFSLGTSASTAYLQINNLKNEDMATYFCARTGTARAFYAMDYWGQGTSVTVSSTKTTAPSVY

SEQ ID NO: 63 - protein, 130 aa, Artificial Sequence
  MIN-D7-1 heavy chain variable region amino acid sequence
EVQLEQSGPELKKPGETVKISCKASGYTFINYGMNWVKQAPGKGLKWMGWINTYTGEPTYVDDFKGRFAFSLETSARTAYLQINNLKNEDMATYFCARTGTTAILNGMDYWGQGTSVTVSSAKTTPPSVY

SEQ ID NO: 64 - protein, 130 aa, Artificial Sequence; identical to SEQ ID NO: 60
  MIN-D7-2 heavy chain variable region amino acid sequence

SEQ ID NO: 65 - protein, 130 aa, Artificial Sequence
  MIN-F2-1 heavy chain variable region amino acid sequence
EVKLEESGPELKKPGETVKISCKASGYTFINYGMNWVKQAPGKGLKWMGWINTYTGEPTYVDDFKGRFAFSLETSARTAYLQINNLKNEDMATYFCARTGTTAILNGMDYWGQGTSVTVSSAKTTPPSVY

SEQ ID NO: 66 - protein, 124 aa, Artificial Sequence
  MIN-F2-2 heavy chain variable region amino acid sequence
EVQLEQSGAELVRPGASVKLSCKALGYTFTDYEMHWVKQTPVHGLEWIGAIHPGSGGTAYNQKFKGKATLTADKSSSTAYMELSSLTSEDSAVYYCTNYGSFAYWGQGTLVTVSAAKTTPPSVY

SEQ ID NO: 67 - protein, 130 aa, Artificial Sequence
  MIN-F2-3 heavy chain variable region amino acid sequence
RCRLQQSGPELKKPGETVKISCKASGYTFINYGMNWVKQAPGKGLKWMGWINTYTGEPTYVDDFKGRFAFSLETSARTAYLQINNLKNEDMATYFCARTGTTAILNGMDYWGQGTSVTVSSAKTTPPSCL

SEQ ID NO: 68 - protein, 130 aa, Artificial Sequence; identical to SEQ ID NO: 63
  MIN-F2-4 heavy chain variable region amino acid sequence

SEQ ID NO: 69 - protein, 113 aa, Artificial Sequence
  MIN-14 light chain variable region amino acid sequence
DIQMTQSPSSLSASLGERVSLTCRASQDIGSSLNWLQQEPDGTIKRLIYATSSLDSGVPKRFSGSRSGSDYSLTISSLESEDFVDYYCLQYASSPHVRCWDQAGAETGCCTNC

SEQ ID NO: 70 - protein, 107 aa, Artificial Sequence
  MIN-17-1 light chain variable region amino acid sequence
DIVLTQSPASLAVSLGQRATISYRASKSVSTSGYSYMHWNQQKPGQPPRLLIYLVSNLESGVPARFSGSGSGTDFTLNIHPVEEEDAATYYCQHIRELTRSEGGPSW

SEQ ID NO: 71 - protein, 115 aa, Artificial Sequence
  MIN-17-2 light chain variable region amino acid sequence
DIQMTQSPASQSASLGESVTITCLASQTIGTWLAWYQQKPGKSPQLLIYAATSLADGVPSRFSGSGSGTKFSFKISSLQAEDFVSYYCQQLYSTPWTFGGGTKLEIKRADAAPTV

SEQ ID NO: 72 - protein, 107 aa, Artificial Sequence; identical to SEQ ID NO: 70
  MIN-29 light chain variable region amino acid sequence

SEQ ID NO: 73 - protein, 107 aa, Artificial Sequence; identical to SEQ ID NO: 70
  MIN-34 light chain variable region amino acid sequence

SEQ ID NO: 74 - protein, 115 aa, Artificial Sequence
  MIN-42 light chain variable region amino acid sequence
DIVMTQSQKFMSTSVGDRVSVTCKASQNVGTNVGWYQQKPGQSPKALIYSASYRYSGVPDRFTGSGSGTDFTLTISNVQSEDLAEYFCQQYNNYPYTFGGGTKLEIKRADAAPTV

SEQ ID NO: 75 - protein, 115 aa, Artificial Sequence
  MIN-45 light chain variable region amino acid sequence
DIQMTQPPASLSASVGETVTITCRASGNIHNFLAWYQQKQGKSPQLLVYNAKTLADGVPSRFSGSGSGTQYSLKINSLQPEDFGSYYCQHFWSTPWTFGGGTKLEIKRADAAPTV

SEQ ID NO: 76 - protein, 105 aa, Artificial Sequence
  MIN-14 heavy chain variable region amino acid sequence
QVQLQQPGAELVKPGASVKLSCKASGYTFTSYWMHWVKQRPGQGLEWIGEINPSNGRTNYNEKFKSKATLTVDKSSSTAYMQLSSLTSEDSAVYYCATYGNYWYF

SEQ ID NO: 77 - protein, 106 aa, Artificial Sequence
  MIN-17-2 heavy chain variable region amino acid sequence
QITLKESGPGIVQPSQPFRLTCTFSGFSLSTSGIGVTWIRQPSGKGLEWLATIWWDDDNRYNPSLKSRLTVSKDTSNNQAFLNIITVETADTAIYYCAQSTMVTAG

SEQ ID NO: 78 - protein, 105 aa, Artificial Sequence; identical to SEQ ID NO: 76
  MIN-17-1 heavy chain variable region amino acid sequence

SEQ ID NO: 79 - protein, 127 aa, Artificial Sequence
  MIN-29 heavy chain variable region amino acid sequence
  misc_feature (12)..(12): Xaa can be any naturally occurring amino acid
DVKLVESGGDLXKLTEGEDIWEGLTLCRDSDQSPLAPVSKPGRVVRPQRSCTVIQGCVLRLQTAHLQVQGVLGIVSGDGESALHSVWIVGATTITINGCDQLQPLLWSLANPRHVIATESESRGCTG

SEQ ID NO: 80 - protein, 104 aa, Artificial Sequence
  MIN-34 heavy chain variable region amino acid sequence
QVQLKQSGPGLVQPSQSLSITCTVSGFSLTSYGVHWVRQSPGKGLEWLGVIWGGGSTDYNAAFISRLSISKDNSKSQVFFKMNSLQANDTAIYYCARNDYPAWF

SEQ ID NO: 81 - protein, 105 aa, Artificial Sequence
  MIN-42 heavy chain variable region amino acid sequence
EVQLVESGGDLVKPGRSLKLSCAASGFTFSSFGMSWVRQTPDKRLEWVATISSGGTYTYYPDSVKGRFTISRDNAKNTLYLQMSSLKSEDTAMYYCSRRFYYDYD

SEQ ID NO: 82 - DNA, 321 bp, Artificial Sequence
  MIN-C2 light chain CL nucleotide sequence
cgggctgatgctgcaccaactgtatccatcttcccaccatccagtgagcagttaacatctggaggtgcctcagtcgtgtgcttcttgaacaacttctaccccaaagacatcaatgtcaagtggaagattgatggcagtgaacgacaaaatggcgtcctgaacagttggactgatcaggacagcaaagacagcacctacagcatgagcagcaccctcacgttgaccaaggacgagtatgaacgacataacagctatacctgtgaggccactcacaagacatcaacttcacccattgtcaagagcttcaacaggaatgagtgt

SEQ ID NO: 83 - DNA, 318 bp, Artificial Sequence
  MIN-C2 Heavy chain CH1 nucleotide sequence
ttcgatgtctggggcgcagggaccacggtcaccgtctcctccgccaaaacgacacccccatctgtctatccactggcccctggatctgctgcccaaactaactccatggtgaccctgggatgcctggtcaagggctatttccctgagccagtgacagtgacctggaactctggatccctgtccagcggtgtgcacaccttcccagctgtcctgcagtctgacctctacactctgagcagctcagtgactgtcccctccagcacctggcccagcgagaccgtcacctgcaacgttgcccacccagccagcaggaccgcg

SEQ ID NO: 84 - protein, 103 aa, Artificial Sequence
  MIN-45 heavy chain variable region amino acid sequence
EVQLQQSGPELVKPGASVKISCKASGYSFTGYFMSWVMQSHGKSLEWIGRINPYNGDTFYNQKFKGKATLTVDKSSTTAHIELRSLASEDSAVYYCARKGLYG

SEQ ID NO: 85 - DNA, 324 bp, Artificial Sequence
  MIN-14 light chain variable region nucleotide sequence
gacatccagatgacccagtctccatcctccttatctgcctctctgggagaaagagtcagtctcacttgtcgagcaagtcaggacattggtagtagcttaaactggcttcagcaggaaccagatggaactattaaacgcctgatctacgccacatccagtttagattctggtgtccccaaaaggttcagtggcagtaggtctgggtcagattattctctcaccatcagcagccttgagtctgaagattttgtagactattactgtctacaatatgctagttctcctcacgttcggtgctgggaccaagctggagctgaaacgggc

SEQ ID NO: 86 - DNA, 323 bp, Artificial Sequence
  MIN-17-1 light chain variable region nucleotide sequence
gacattgtgctgacacagtctcctgcttccttagctgtatctctggggcagagggccaccatctcatacagggccagcaaaagtgtcagtacatctggctatagttatatgcactggaaccaacagaaaccaggacagccacccagactcctcatctatcttgtatccaacctagaatctggggtccctgccaggttcagtggcagtgggtctgggacagacttcaccctcaacatccatcctgtggaggaggaggatgctgcaacctattactgtcagcacattagggagcttacacgttcggaggggggaccaagctggaa

SEQ ID NO: 87 - DNA, 345 bp, Artificial Sequence
  MIN-17-2 light chain variable region nucleotide sequence
gacattcagatgacccagtctcctgcctcccagtctgcatctctgggagaaagtgtcaccatcacatgcctggcaagtcagaccattggtacatggttagcatggtatcagcagaaaccagggaaatctcctcagctcctgatttatgctgcaaccagcttggcagatggggtcccatcaaggttcagtggtagtggatctggcacaaaattttctttcaagatcagcagcctacaggctgaagattttgtaagttattactgtcaacaactttacagtactccgtggacgttcggtggaggcaccaagctggaaatcaaacgggctgatgctgcaccaactgta

SEQ ID NO: 88 - DNA, 323 bp, Artificial Sequence
  MIN-29 light chain variable region nucleotide sequence
gtgacattgtgctgacacagtctcctgcttccttagctgtatctctggggcagagggccaccatctcatacagggccagcaaaagtgtcagtacatctggctatagttatatgcactggaaccaacagaaaccaggacagccacccagactcctcatctatcttgtatccaacctagaatctggggtccctgccaggttcagtggcagtgggtctgggacagacttcaccctcaacatccatcctgtggaggaggaggatgctgcaacctattactgtcagcacattagggagcttacacgttcggaggggggaccaagctgg

SEQ ID NO: 89 - DNA, 321 bp, Artificial Sequence
  MIN-34 light chain variable region nucleotide sequence
gacattgtgctgacacagtctcctgcttccttagctgtatctctggggcagagggccaccatctcatacagggccagcaaaagtgtcagtacatctggctatagttatatgcactggaaccaacagaaaccaggacagccacccagactcctcatctatcttgtatccaacctagaatctggggtccctgccaggttcagtggcagtgggtctgggacagacttcaccctcaacatccatcctgtggaggaggaggatgctgcaacctattactgtcagcacattagggagcttacacgttcggaggggggaccaagctgg

SEQ ID NO: 90 - DNA, 345 bp, Artificial Sequence
  MIN-42 light chain variable region nucleotide sequence
gacattgtgatgacccagtctcaaaaattcatgtccacatcagtaggagacagggtcagcgtcacctgcaaggccagtcagaatgtgggtactaatgtaggttggtatcaacagaaaccagggcaatctcctaaagcactgatttactcggcatcctaccggtacagtggagtccctgatcgcttcacaggcagtggatctgggacagatttcactctcaccatcagcaatgtgcagtctgaagacttggcagagtatttctgtcagcaatataacaactatccgtacacgttcggaggggggaccaagctggaaataaaacgggctgatgctgcaccaactgta

SEQ ID NO: 91 - DNA, 345 bp, Artificial Sequence
  MIN-45 light chain variable region nucleotide sequence
gacatccagatgactcagcctccagcctccctatctgcatctgtgggagaaactgtcaccatcacatgtcgagcaagtgggaatattcacaattttttagcatggtatcagcagaaacagggaaaatctcctcagctcctggtctataatgcaaaaaccttagcagatggtgtgccatcaaggttcagtggcagtggatcaggaacacaatattctctcaagatcaacagcctgcagcctgaagattttgggagttattactgtcaacatttttggagtactccgtggacgttcggtggaggcaccaagctggaaatcaaacgggctgatgctgcaccaactgta

SEQ ID NO: 92 - DNA, 315 bp, Artificial Sequence
  MIN-14 heavy chain variable region nucleotide sequence
caggtccaactgcagcagcctggggctgaactggtgaagcctggggcttcagtgaagctgtcctgcaaggcttctggctacaccttcaccagctactggatgcactgggtgaagcagaggcctggacaaggccttgagtggattggagagattaatcctagcaacggtcgtactaactacaatgagaagttcaagagcaaggccacactgactgtagacaaatcctccagcacagcctacatgcaactcagcagcctgacatctgaggactctgcggtctattactgtgcaacctatggtaactactggtacttc

SEQ ID NO: 93 - DNA, 315 bp, Artificial Sequence; identical to SEQ ID NO: 92
  MIN-17-1 heavy chain variable region nucleotide sequence

SEQ ID NO: 94 - DNA, 318 bp, Artificial Sequence
  MIN-17-2 heavy chain variable region nucleotide sequence
cagattactctgaaagagtctggccctgggatagttcagccatcccagcccttcagacttacttgcactttctctgggttttcactgagcacttctggtataggtgtaacctggattcgtcagccctcagggaaaggtctggagtggctggcaacgatttggtgggatgatgataaccgctacaacccatctctaaagagcaggctcacagtctccaaagacacctccaacaaccaagcattcctgaatatcatcactgtggaaactgcagatactgccatatactactgtgctcagtctactatggttacggcggga

SEQ ID NO: 95 - DNA, 313 bp, Artificial Sequence
  MIN-34 heavy chain variable region nucleotide sequence
ccaggtgcagctgaagcagtcaggacctggcctagtgcagccctcacagagcctgtccatcacctgcacagtctctggtttctcattaactagctatggtgtacactgggttcgccagtctccaggaaagggtctggagtggctgggagtgatatggggtggtggaagcacagactataatgcagctttcatatccagactgagcatcagcaaggacaattccaagagccaagttttctttaaaatgaacagtctgcaagctaatgacacagccatatattactgtgccagaaatgactatccggcctggttt

SEQ ID NO: 96 - DNA, 317 bp, Artificial Sequence
  MIN-42 heavy chain variable region nucleotide sequence
gtgaggtgcaactggtggagtctgggggagacttagtgaagcctggaaggtccctgaaactctcctgtgcagcctctggattcactttcagtagctttggcatgtcttgggttcgccagactccagacaagaggctggagtgggtcgcaaccattagtagtggtggtacttacacctactatccagacagtgtgaaggggcgattcaccatctccagagacaatgccaagaacaccctgtacctgcaaatgagcagtctgaagtctgaggacacagccatgtattactgttcaagaaggttctactatgattacgac

SEQ ID NO: 97 - DNA, 309 bp, Artificial Sequence
  MIN-45 heavy chain variable region nucleotide sequence
gaggttcagctgcagcagtctggacctgagctggtgaagcctggggcttcagtgaagatatcctgcaaggcttctggttactcatttactggctactttatgagctgggtgatgcagagccatggaaagagccttgagtggattggacgtattaatccttacaatggtgatactttctacaaccagaagttcaagggcaaggccacattgactgtagacaaatcctctaccacagcccacatagagctccggagcctggcatctgaggactctgcagtctattattgtgcaagaaagggcctctatggg

SEQ ID NO: 98 - protein, 23 aa, Artificial Sequence
  MIN-C2 light chain variable framework region 1 (FWR1) amino acid sequence
DIVITQSTASLGVSLGQRATISC

SEQ ID NO: 99 - protein, 23 aa, Artificial Sequence
  MIN-E6 light chain variable framework region 1 (FWR1) amino acid sequence
DIVITQTTAIMSASPGEEVTLTC

SEQ ID NO: 100 - protein, 23 aa, Artificial Sequence
  MIN-A2-1 light chain variable framework region 1 (FWR1) amino acid sequence
DIVLTQSTEIMSASPGEKVTITC

SEQ ID NO: 101 - protein, 23 aa, Artificial Sequence
  MIN-A2-2 light chain variable framework region 1 (FWR1) amino acid sequence
DIVMTQSPAIMSASPGEKVTMTC

SEQ ID NO: 102 - protein, 23 aa, Artificial Sequence
  MIN-C9-1 light chain variable framework region 1 (FWR1) amino acid sequence
DIVLTQTTAIMSASPGEKVTITC

SEQ ID NO: 103 - protein, 23 aa, Artificial Sequence
  MIN-C9-2 light chain variable framework region 1 (FWR1) amino acid sequence
DIVITQSTAIMSASPGEKVTITC

SEQ ID NO: 104 - protein, 23 aa, Artificial Sequence
  MIN-D7-1 light chain variable framework region 1 (FWR1) amino acid sequence
DIVITQTPAIMSASPGEKVTMTC

SEQ ID NO: 105 - protein, 23 aa, Artificial Sequence
  MIN-D7-2 light chain variable framework region 1 (FWR1) amino acid sequence
DIVLTQSTAIMSASPGEKVTMTC

SEQ ID NO: 106 - protein, 23 aa, Artificial Sequence
  MIN-F2-1 light chain variable framework region 1 (FWR1) amino acid sequence
DIVMTQSPEIMSASPGEKVTITC

SEQ ID NO: 107 - protein, 23 aa, Artificial Sequence
  MIN-F2-2 light chain variable framework region 1 (FWR1) amino acid sequence
DIVITQSTEIMSASPGEKVTITC

SEQ ID NO: 108 - protein, 15 aa, Artificial Sequence
  MIN-C2 light chain variable complementarity determining region 1 (CDR1) amino acid sequence
RASKSVSTSGYSYMH

SEQ ID NO: 109 - protein, 10 aa, Artificial Sequence
  MIN-E6 light chain variable complementarity determining region 1 (CDR1) amino acid sequence
SATSSVSYIH

SEQ ID NO: 110 - protein, 10 aa, Artificial Sequence
  MIN-A2-1 light chain variable complementarity determining region 1 (CDR1) amino acid sequence
SASSSISYIH

SEQ ID NO: 111 - skipped
  000

SEQ ID NO: 112 - protein, 10 aa, Artificial Sequence
  MIN-A2-2 light chain variable complementarity determining region 1 (CDR1) amino acid sequence
SASSSVSYMH

SEQ ID NO: 113 - protein, 10 aa, Artificial Sequence
  MIN-C9-1 light chain variable complementarity determining region 1 (CDR1) amino acid sequence
SASSSVSYMY

SEQ ID NO: 114 - protein, 10 aa, Artificial Sequence
  MIN-C9-2 light chain variable complementarity determining region 1 (CDR1) amino acid sequence
SASSSVSYTY

SEQ ID NO: 115 - protein, 10 aa, Artificial Sequence
  MIN-D7-1 light chain variable complementarity determining region 1 (CDR1) amino acid sequence
SASSSVSYMH

SEQ ID NO: 116 - protein, 10 aa, Artificial Sequence
  MIN-D7-2 light chain variable complementarity determining region 1 (CDR1) amino acid sequence
SASSSVSYMH

SEQ ID NO: 117 - protein, 10 aa, Artificial Sequence
  MIN-F2-1 light chain variable complementarity determining region 1 (CDR1) amino acid sequence
SASSSISYIH

SEQ ID NO: 118 - protein, 10 aa, Artificial Sequence
  MIN-F2-2 light chain variable complementarity determining region 1 (CDR1) amino acid sequence
SASSSISYIH

SEQ ID NO: 119 - protein, 15 aa, Artificial Sequence
  MIN-C2 light chain variable framework region 2 (FWR2) amino acid sequence
WYQQRPGQPPKLLIY

SEQ ID NO: 120 - protein, 15 aa, Artificial Sequence
  MIN-E6 light chain variable framework region 2 (FWR2) amino acid sequence
WFQQRPGTSPKLWIY

SEQ ID NO: 121 - protein, 15 aa, Artificial Sequence
  MIN-A2-1 light chain variable framework region 2 (FWR2) amino acid sequence
WFQQKPGTSPKLWIF

SEQ ID NO: 122 - protein, 15 aa, Artificial Sequence
  MIN-A2-2 light chain variable framework region 2 (FWR2) amino acid sequence
WFQQKPGTSPKLWIY

SEQ ID NO: 123 - protein, 15 aa, Artificial Sequence
  MIN-C9-1 light chain variable framework region 2 (FWR2) amino acid sequence
WFQQKPGTSPKLWIY

SEQ ID NO: 124 - protein, 15 aa, Artificial Sequence
  MIN-C9-2 light chain variable framework region 2 (FWR2) amino acid sequence
WFQQKPGTSPKLWIY

SEQ ID NO: 125 - protein, 15 aa, Artificial Sequence
  MIN-D7-1 light chain variable framework region 2 (FWR2) amino acid sequence
WFQQKPGTSPKLWIY

SEQ ID NO: 126 - protein, 15 aa, Artificial Sequence
  MIN-D7-2 light chain variable framework region 2 (FWR2) amino acid sequence
WFQQKPGTSPKLWIY

SEQ ID NO: 127 - protein, 15 aa, Artificial Sequence
  MIN-F2-1 light chain variable framework region 2 (FWR2) amino acid sequence
WFQQKPGTSPKLWIF

SEQ ID NO: 128 - protein, 15 aa, Artificial Sequence
  MIN-F2-2 light chain variable framework region 2 (FWR2) amino acid sequence
WFQQKPGTSPKLWIF

SEQ ID NO: 129 - protein, 7 aa, Artificial Sequence
  MIN-C2 light chain variable complementarity determining region 2 (CDR2) amino acid sequence
LASNLES

SEQ ID NO: 130 - protein, 7 aa, Artificial Sequence
  MIN-E6 light chain variable complementarity determining region 2 (CDR2) amino acid sequence
STSNLAS

SEQ ID NO: 131 - protein, 7 aa, Artificial Sequence
  MIN-A2-1 light chain variable complementarity determining region 2 (CDR2) amino acid sequence
GTSNLAS

SEQ ID NO: 132 - protein, 7 aa, Artificial Sequence
  MIN-A2-2 light chain variable complementarity determining region 2 (CDR2) amino acid sequence
STSNLAS

SEQ ID NO: 133 - protein, 7 aa, Artificial Sequence
  MIN-C9-1 light chain variable complementarity determining region 2 (CDR2) amino acid sequence
STSNLAS

SEQ ID NO: 134 - protein, 7 aa, Artificial Sequence
  MIN-C9-2 light chain variable complementarity determining region 2 (CDR2) amino acid sequence
STSNLAS

SEQ ID NO: 135 - protein, 7 aa, Artificial Sequence
  MIN-D7-1 light chain variable complementarity determining region 2 (CDR2) amino acid sequence
STSNLAS

SEQ ID NO: 136 - protein, 7 aa, Artificial Sequence
  MIN-D7-2 light chain variable complementarity determining region 2 (CDR2) amino acid sequence
STSNLAS

SEQ ID NO: 137 - protein, 7 aa, Artificial Sequence
  MIN-F2-1 light chain variable complementarity determining region 2 (CDR2) amino acid sequence
GTSNLAS

SEQ ID NO: 138 - protein, 7 aa, Artificial Sequence
  MIN-F2-2 light chain variable complementarity determining region 2 (CDR2) amino acid sequence
GTSNLAS

SEQ ID NO: 139 - protein, 32 aa, Artificial Sequence
  MIN-C2 light chain variable framework region 3 (FWR3) amino acid sequence
GVPARFSGSGSGTDFTLNIHPVEEEDAATYYC

SEQ ID NO: 140 - protein, 32 aa, Artificial Sequence
  MIN-E6 light chain variable framework region 3 (FWR3) amino acid sequence
GVPVRFSGSGYGTSYSLTISRMEAEDAATYYC

SEQ ID NO: 141 - protein, 32 aa, Artificial Sequence
  MIN-A2-1 light chain variable framework region 3 (FWR3) amino acid sequence
GVPARFSGSGSGTSYSLTVSRMEAEDTATYYC

SEQ ID NO: 142 - protein, 32 aa, Artificial Sequence
  MIN-A2-2 light chain variable framework region 3 (FWR3) amino acid sequence
GAPARFSGSGSGTSYSLTVSRMESEDAATYYC

SEQ ID NO: 143 - protein, 32 aa, Artificial Sequence
  MIN-C9-1 light chain variable framework region 3 (FWR3) amino acid sequence
GVPARFSGSGSGTSYSLTISRMEAEDAATYYC

SEQ ID NO: 144 - protein, 32 aa, Artificial Sequence; identical to SEQ ID NO: 143
  MIN-C9-2 light chain variable framework region 3 (FWR3) amino acid sequence

SEQ ID NO: 145 - protein, 32 aa, Artificial Sequence
  MIN-D7-1 light chain variable framework region 3 (FWR3) amino acid sequence
GVPARFSGSGSGTSYSLTVSRMESEDAATYYC

SEQ ID NO: 146 - protein, 32 aa, Artificial Sequence; identical to SEQ ID NO: 145
  MIN-D7-2 light chain variable framework region 2 (FWR2) amino acid sequence

SEQ ID NO: 147 - protein, 32 aa, Artificial Sequence; identical to SEQ ID NO: 141
  MIN-F2-1 light chain variable framework region 3 (FWR3) amino acid sequence

SEQ ID NO: 148 - protein, 32 aa, Artificial Sequence; identical to SEQ ID NO: 141
  MIN-F2-2 light chain variable framework region 3 (FWR3) amino acid sequence

SEQ ID NO: 149 - protein, 9 aa, Artificial Sequence
  MIN-C2 light chain variable complementarity determining region 3 (CDR3) amino acid sequence
QHSRELPFT

SEQ ID NO: 150 - protein, 9 aa, Artificial Sequence
  MIN-E6 light chain variable complementarity determining region 3 (CDR3) amino acid sequence
QQRSSSPFT

SEQ ID NO: 151 - protein, 9 aa, Artificial Sequence
  MIN-A2-1 light chain variable complementarity determining region 3 (CDR3) amino acid sequence
QQRSNYPFT

SEQ ID NO: 152 - protein, 9 aa, Artificial Sequence
  MIN-A2-2 light chain variable complementarity determining region 3 (CDR3) amino acid sequence
QQRSSYPST

SEQ ID NO: 153 - protein, 9 aa, Artificial Sequence
  MIN-C9-1 light chain variable complementarity determining region 3 (CDR3) amino acid sequence
QQRSSYPST

SEQ ID NO: 154 - protein, 9 aa, Artificial Sequence
  MIN-C9-2 light chain variable complementarity determining region 3 (CDR3) amino acid sequence
QQRSSYPST

SEQ ID NO: 155 - protein, 9 aa, Artificial Sequence
  MIN-D7-1 light chain variable complementarity determining region 3 (CDR3) amino acid sequence
QQRSSYPST

SEQ ID NO: 156 - protein, 9 aa, Artificial Sequence
  MIN-D7-2 light chain variable complementarity determining region 3 (CDR3) amino acid sequence
QQRSSYPST

SEQ ID NO: 157 - protein, 9 aa, Artificial Sequence
  MIN-F2-1 light chain variable complementarity determining region 3 (CDR3) amino acid sequence
QQRSNYPFT

SEQ ID NO: 158 - protein, 9 aa, Artificial Sequence
  MIN-F2-2 light chain variable complementarity determining region 3 (CDR3) amino acid sequence
QQRSNYPFT

SEQ ID NO: 159 - protein, 30 aa, Artificial Sequence
  MIN-C2 heavy chain variable framework region 1 (FWR1) amino acid sequence
EVQLEESGGGLVKPGGSLKLSCAASGFTFS

SEQ ID NO: 160 - protein, 30 aa, Artificial Sequence
  MIN-E6-7 heavy chain variable framework region 1 (FWR1) amino acid sequence
EVKLEESGGDLVKPGGSLKLSCAASGFTFS

SEQ ID NO: 161 - protein, 30 aa, Artificial Sequence
  MIN-E6-8 heavy chain variable framework region 1 (FWR1) amino acid sequence
EVKLEESGGDLVKPGGSLKLSCVVSGFTFS

SEQ ID NO: 162 - protein, 30 aa, Artificial Sequence
  MIN-A2-1 heavy chain variable framework region 1 (FWR1) amino acid sequence
EVKLQESGPELKKPGETVEISCKASGYTFT

SEQ ID NO: 163 - protein, 30 aa, Artificial Sequence
  MIN-A2-2 heavy chain variable framework region 1 (FWR1) amino acid sequence
EVQLQQSGPELKKPGETVKISCKASGYTFT

SEQ ID NO: 164 - protein, 30 aa, Artificial Sequence
  MIN-C9-1 heavy chain variable framework region 1 (FWR1) amino acid sequence
QVQLQESGPELKQPGETVKISCKASGYTFT

SEQ ID NO: 165 - protein, 30 aa, Artificial Sequence
  MIN-C9-2 heavy chain variable framework region 1 (FWR1) amino acid sequence
QVQLQQSGPELKQPGETVKISCKASGYTFT

SEQ ID NO: 166 - protein, 30 aa, Artificial Sequence
  MIN-D7-1 heavy chain variable framework region 1 (FWR1) amino acid sequence
EVQLEQSGPELKKPGETVKISCKASGYTFI

SEQ ID NO: 167 - protein, 30 aa, Artificial Sequence; identical to SEQ ID NO: 163
  MIN-D7-2 heavy chain variable framework region 1 (FWR1) amino acid sequence

SEQ ID NO: 168 - protein, 30 aa, Artificial Sequence
  MIN-F2-1 heavy chain variable framework region 1 (FWR1) amino acid sequence
EVKLEESGPELKKPGETVKISCKASGYTFI

SEQ ID NO: 169 - protein, 30 aa, Artificial Sequence
  MIN-F2-2 heavy chain variable framework region 1 (FWR1) amino acid sequence
EVQLEQSGAELVRPGASVKLSCKALGYTFT

SEQ ID NO: 170 - protein, 30 aa, Artificial Sequence
  MIN-F2-3 heavy chain variable framework region 1 (FWR1) amino acid sequence
RCRLQQSGPELKKPGETVKISCKASGYTFI

SEQ ID NO: 171 - protein, 30 aa, Artificial Sequence; identical to SEQ ID NO: 166
  MIN-F2-4 heavy chain variable framework region 1 (FWR1) amino acid sequence

SEQ ID NO: 172 - protein, 5 aa, Artificial Sequence
  MIN-C2 heavy chain variable complementarity determining region 1 (CDR1) amino acid sequence
GYAMS

SEQ ID NO: 173 - protein, 5 aa, Artificial Sequence
  MIN-E6-7 heavy chain variable complementarity determining region 1 (CDR1) amino acid sequence
RYGMS

SEQ ID NO: 174 - protein, 5 aa, Artificial Sequence
  MIN-E6-8 heavy chain variable complementarity determining region 1 (CDR1) amino acid sequence
RYGMS

SEQ ID NO: 175 - protein, 5 aa, Artificial Sequence
  MIN-A2-1 heavy chain variable complementarity determining region 1 (CDR1) amino acid sequence
NYGMN

SEQ ID NO: 176 - protein, 5 aa, Artificial Sequence
  MIN-A2-2 heavy chain variable complementarity determining region 1 (CDR1) amino acid sequence
NYGMN

SEQ ID NO: 177 - protein, 5 aa, Artificial Sequence
  MIN-C9-1 heavy chain variable complementarity determining region 1 (CDR1) amino acid sequence
NNGMN

SEQ ID NO: 178 - protein, 5 aa, Artificial Sequence
  MIN-C9-2 heavy chain variable complementarity determining region 1 (CDR1) amino acid sequence
NNGMN

SEQ ID NO: 179 - protein, 5 aa, Artificial Sequence
  MIN-D7-1 heavy chain variable complementarity determining region 1 (CDR1) amino acid sequence
NYGMN

SEQ ID NO: 180 - protein, 5 aa, Artificial Sequence
  MIN-D7-2 heavy chain variable complementarity determining region 1 (CDR1) amino acid sequence
NYGMN

SEQ ID NO: 181 - protein, 5 aa, Artificial Sequence
  MIN-F2-1 heavy chain variable complementarity determining region 1 (CDR1) amino acid sequence
NYGMN

SEQ ID NO: 182 - protein, 5 aa, Artificial Sequence
  MIN-F2-2 heavy chain variable complementarity determining region 1 (CDR1) amino acid sequence
DYEMH

SEQ ID NO: 183 - protein, 5 aa, Artificial Sequence
  MIN-F2-3 heavy chain variable complementarity determining region 1 (CDR1) amino acid sequence
NYGMN

SEQ ID NO: 184 - protein, 5 aa, Artificial Sequence
  MIN-F2-4 heavy chain variable complementarity determining region 1 (CDR1) amino acid sequence
NYGMN

SEQ ID NO: 185 - protein, 14 aa, Artificial Sequence
  MIN-C2 heavy chain variable framework region 2 (FWR2) amino acid sequence
WVRQTPEKRLEWVA

SEQ ID NO: 186 - protein, 14 aa, Artificial Sequence
  MIN-E6-7 heavy chain variable framework region 2 (FWR2) amino acid sequence
WVRQTPDKRLEWVA

SEQ ID NO: 187 - protein, 14 aa, Artificial Sequence
  MIN-E6-8 heavy chain variable framework region 2 (FWR2) amino acid sequence
WVRQTPGKRLEWVA

SEQ ID NO: 188 - protein, 14 aa, Artificial Sequence
  MIN-A2-1 heavy chain variable framework region 2 (FWR2) amino acid sequence
WVKQAPGKGLKWMG

SEQ ID NO: 189 - protein, 14 aa, Artificial Sequence
  MIN-A2-2 heavy chain variable framework region 2 (FWR2) amino acid sequence
WVKQAPGKGLKWMG

SEQ ID NO: 190 - protein, 14 aa, Artificial Sequence
  MIN-C9-1 heavy chain variable framework region 2 (FWR2) amino acid sequence
WVKQAPGKGLKWMG

SEQ ID NO: 191 - protein, 14 aa, Artificial Sequence
  MIN-C9-2 heavy chain variable framework region 2 (FWR2) amino acid sequence
WVKQAPGKGLKWMG

SEQ ID NO: 192 - protein, 14 aa, Artificial Sequence
  MIN-D7-1 heavy chain variable framework region 2 (FWR2) amino acid sequence
WVKQAPGKGLKWMG

SEQ ID NO: 193 - protein, 14 aa, Artificial Sequence
  MIN-D7-2 heavy chain variable framework region 2 (FWR2) amino acid sequence
WVKQAPGKGLKWMG

SEQ ID NO: 194 - protein, 14 aa, Artificial Sequence
  MIN-F2-1 heavy chain variable framework region 2 (FWR2) amino acid sequence
WVKQAPGKGLKWMG

SEQ ID NO: 195 - protein, 14 aa, Artificial Sequence
  MIN-F2-2 heavy chain variable framework region 2 (FWR2) amino acid sequence
WVKQTPVHGLEWIG

SEQ ID NO: 196 - protein, 14 aa, Artificial Sequence
  MIN-F2-3 heavy chain variable framework region 2 (FWR2) amino acid sequence
WVKQAPGKGLKWMG

SEQ ID NO: 197 - protein, 14 aa, Artificial Sequence
  MIN-F2-4 heavy chain variable framework region 2 (FWR2) amino acid sequence
WVKQAPGKGLKWMG

SEQ ID NO: 198 - protein, 17 aa, Artificial Sequence
  MIN-C2 heavy chain variable complementarity determining region 2 (CDR2) amino acid sequence
TISSGGTYIYYPDSVKG

SEQ ID NO: 199 - protein, 17 aa, Artificial Sequence
  MIN-E6-7 heavy chain variable complementarity determining region 2 (CDR2) amino acid sequence
TISSGGTYIYYPDSVKG

SEQ ID NO: 200 - protein, 17 aa, Artificial Sequence
  MIN-E6-8 heavy chain variable complementarity determining region 2 (CDR2) amino acid sequence
TISGGGTYIYYPDSVKG

SEQ ID NO: 201 - protein, 17 aa, Artificial Sequence
  MIN-A2-1 heavy chain variable complementarity determining region 2 (CDR2) amino acid sequence
WINTYTGEPTYAGDFKG

SEQ ID NO: 202 - protein, 17 aa, Artificial Sequence
  MIN-A2-2 heavy chain variable complementarity determining region 2 (CDR2) amino acid sequence
WINTYTGEPTYAGDFKG

SEQ ID NO: 203 - protein, 17 aa, Artificial Sequence
  MIN-C9-1 heavy chain variable complementarity determining region 2 (CDR2) amino acid sequence
WINTYTGEPTYADDFKG

SEQ ID NO: 204 - protein, 17 aa, Artificial Sequence
  MIN-C9-2 heavy chain variable complementarity determining region 2 (CDR2) amino acid sequence
WINTYTGEPTYADDFKG

SEQ ID NO: 205 - protein, 17 aa, Artificial Sequence
  MIN-D7-1 heavy chain variable complementarity determining region 2 (CDR2) amino acid sequence
WINTYTGEPTYVDDFKG

SEQ ID NO: 206 - protein, 17 aa, Artificial Sequence
  MIN-D7-2 heavy chain variable complementarity determining region 2 (CDR2) amino acid sequence
WINTYTGEPTYAGDFKG

SEQ ID NO: 207 - protein, 17 aa, Artificial Sequence
  MIN-F2-1 heavy chain variable complementarity determining region 2 (CDR2) amino acid sequence
WINTYTGEPTYVDDFKG

SEQ ID NO: 208 - protein, 17 aa, Artificial Sequence
  MIN-F2-2 heavy chain variable complementarity determining region 2 (CDR2) amino acid sequence
AIHPGSGGTAYNQKFKG

SEQ ID NO: 209 - protein, 17 aa, Artificial Sequence
  MIN-F2-3 heavy chain variable complementarity determining region 2 (CDR2) amino acid sequence
WINTYTGEPTYVDDFKG

SEQ ID NO: 210 - protein, 17 aa, Artificial Sequence
  MIN-F2-4 heavy chain variable complementarity determining region 2 (CDR2) amino acid sequence
WINTYTGEPTYVDDFKG

SEQ ID NO: 211 - protein, 32 aa, Artificial Sequence
  MIN-C2 heavy chain variable framework region 3 (FWR3) amino acid sequence
RFTISRDNAKNTLYLQMSSLRSEDTAMYYCAR

SEQ ID NO: 212 - protein, 32 aa, Artificial Sequence
  MIN-E6-7 heavy chain variable framework region 3 (FWR3) amino acid sequence
RFTISRDNAKNTLYLQMSSLKSEDTAMYYCAR

SEQ ID NO: 213 - protein, 32 aa, Artificial Sequence
  MIN-E6-8 heavy chain variable framework region 3 (FWR3) amino acid sequence
RFTISRDNAKNTLYLQMSSLKSEDTAMYHCTR

SEQ ID NO: 214 - protein, 32 aa, Artificial Sequence
  MIN-A2-1 heavy chain variable framework region 3 (FWR3) amino acid sequence
RFAFSLETSASTAYLQINTLKNEDTATYFCAR

SEQ ID NO: 215 - protein, 32 aa, Artificial Sequence; identical to SEQ ID NO: 214
  MIN-A2-2 heavy chain variable framework region 3 (FWR3) amino acid sequence

SEQ ID NO: 216 - protein, 32 aa, Artificial Sequence
  MIN-C9-1 heavy chain variable framework region 3 (FWR3) amino acid sequence
RFAFSLDTSASTAYLQINNLKNEDMATYFCAR

SEQ ID NO: 217 - protein, 32 aa, Artificial Sequence
  MIN-C9-2 heavy chain variable framework region 3 (FWR3) amino acid sequence
RFAFSLGTSASTAYLQINNLKNEDMATYFCAR

SEQ ID NO: 218 - protein, 32 aa, Artificial Sequence
  MIN-D7-1 heavy chain variable framework region 3 (FWR3) amino acid sequence
RFAFSLETSARTAYLQINNLKNEDMATYFCAR

SEQ ID NO: 219 - protein, 32 aa, Artificial Sequence; identical to SEQ ID NO: 214
  MIN-D7-2 heavy chain variable framework region 3 (FWR3) amino acid sequence

SEQ ID NO: 220 - protein, 32 aa, Artificial Sequence; identical to SEQ ID NO: 218
  MIN-F2-1 heavy chain variable framework region 3 (FWR3) amino acid sequence

SEQ ID NO: 221 - protein, 32 aa, Artificial Sequence
  MIN-F2-2 heavy chain variable framework region 3 (FWR3) amino acid sequence
KATLTADKSSSTAYMELSSLTSEDSAVYYCTN

SEQ ID NO: 222 - protein, 32 aa, Artificial Sequence; identical to SEQ ID NO: 218
  MIN-F2-3 heavy chain variable framework region 3 (FWR3) amino acid sequence

SEQ ID NO: 223 - protein, 32 aa, Artificial Sequence; identical to SEQ ID NO: 218
  MIN- F2-4 heavy chain variable framework region 3 (FWR3) amino acid sequence

SEQ ID NO: 224 - protein, 9 aa, Artificial Sequence
  MIN-C2 heavy chain variable complementarity determining region 3 (CDR3) amino acid sequence
LGGDNYYEY

SEQ ID NO: 225 - protein, 10 aa, Artificial Sequence
  MIN-E6-7 heavy chain variable complementarity determining region 3 (CDR3) amino acid sequence
DNYGSSYDYA

SEQ ID NO: 226 - protein, 10 aa, Artificial Sequence
  MIN-E6-8 heavy chain variable complementarity determining region 3 (CDR3) amino acid sequence
DNYGRNYDYG

SEQ ID NO: 227 - protein, 9 aa, Artificial Sequence
  MIN-A2-1 heavy chain variable complementarity determining region 3 (CDR3) amino acid sequence
SGDGYWYYA

SEQ ID NO: 228 - protein, 9 aa, Artificial Sequence
  MIN- A2-2 heavy chain variable complementarity determining region 3 (CDR3) amino acid sequence
SGDGYWYYA

SEQ ID NO: 229 - protein, 9 aa, Artificial Sequence
  MIN-C9-1 heavy chain variable complementarity determining region 3 (CDR3) amino acid sequence
TGTARAFYA

SEQ ID NO: 230 - protein, 9 aa, Artificial Sequence
  MIN-C9-2  heavy chain variable complementarity determining region 3 (CDR3) amino acid sequence
TGTARAFYA

SEQ ID NO: 231 - protein, 9 aa, Artificial Sequence
  MIN-D7-1 heavy chain variable complementarity determining region 3(CDR3) amino acid sequence
TGTTAILNG

SEQ ID NO: 232 - protein, 9 aa, Artificial Sequence
  MIN-D7-2 heavy chain variable complementarity determining region3 (CDR3) amino acid sequence
SGDGYWYYA

SEQ ID NO: 233 - protein, 9 aa, Artificial Sequence
  MIN-F2-1 heavy chain variable complementarity determining region 3 (CDR3 ) amino acid sequence
TGTTAILNG

SEQ ID NO: 234 - protein, 5 aa, Artificial Sequence
  MIN-F2-2 heavy chain variable complementarity determining region 3(CDR3) amino acid sequence
YGSFA

SEQ ID NO: 235 - protein, 9 aa, Artificial Sequence
  MIN-F2-3 heavy chain variable complementarity determining region 3 (CDR3) amino acid sequence
TGTTAILNG

SEQ ID NO: 236 - protein, 9 aa, Artificial Sequence
  MIN-F2-4 heavy chain variable complementarity determining region 3(CDR3) amino acid sequence
TGTTAILNG

SEQ ID NO: 237 - protein, 23 aa, Artificial Sequence
  MIN-14 light chain variable framework region 1 (FWR1) amino acid sequence
DIQMTQSPSSLSASLGERVSLTC

SEQ ID NO: 238 - protein, 23 aa, Artificial Sequence
  MIN-17-1 light chain variable framework region 1 (FWR1) amino acid sequence
DIVLTQSPASLAVSLGQRATISY

SEQ ID NO: 239 - protein, 23 aa, Artificial Sequence
  MIN-17-2 light chain variable framework region 1 (FWR1) amino acid sequence
DIQMTQSPASQSASLGESVTITC

SEQ ID NO: 240 - protein, 23 aa, Artificial Sequence
  MIN-29 light chain variable framework region 1 (FWR1) amino acid sequence
DIVLTQSPASLAVSLGQRATISY

SEQ ID NO: 241 - protein, 23 aa, Artificial Sequence
  MIN-34 light chain variable framework region 1 (FWR1) amino acid sequence
DIVLTQSPASLAVSLGQRATISY

SEQ ID NO: 242 - protein, 23 aa, Artificial Sequence
  MIN-42 light chain variable framework region 1 (FWR1) amino acid sequence
DIVMTQSQKFMSTSVGDRVSVTC

SEQ ID NO: 243 - protein, 23 aa, Artificial Sequence
  MIN- 45 light chain variable framework region 1 (FWR1) amino acid sequence
DIQMTQPPASLSASVGETVTITC

SEQ ID NO: 244 - protein, 11 aa, Artificial Sequence
  MIN- 14 light chain variable complementarity determining region 1 (CDR1) amino acid sequence
RASQDIGSSLN

SEQ ID NO: 245 - protein, 15 aa, Artificial Sequence
  MIN- 17-1 light chain variable complementarity determining region 1 (CDR1) amino acid sequence
RASKSVSTSGYSYMH

SEQ ID NO: 246 - protein, 11 aa, Artificial Sequence
  MIN- 17-2 light chain variable complementarity determining region 1 (CDR1) amino acid sequence
LASQTIGTWLA

SEQ ID NO: 247 - protein, 15 aa, Artificial Sequence
  MIN- 29 light chain variable complementarity determining region 1 (CDR1) amino acid sequence
RASKSVSTSGYSYMH

SEQ ID NO: 248 - protein, 15 aa, Artificial Sequence
  MIN- 34 light chain variable complementarity determining region 1 (CDR1) amino acid sequence
RASKSVSTSGYSYMH

SEQ ID NO: 249 - protein, 11 aa, Artificial Sequence
  MIN- 42 light chain variable complementarity determining region 1 (CDR1) amino acid sequence
KASQNVGTNVG

SEQ ID NO: 250 - protein, 11 aa, Artificial Sequence
  MIN-45 light chain variable complementarity determining region 1 (CDR1) amino acid sequence
RASGNIHNFLA

SEQ ID NO: 251 - protein, 15 aa, Artificial Sequence
  MIN-14 light chain variable framework region 2 (FWR2) amino acid sequence
WLQQEPDGTIKRLIY

SEQ ID NO: 252 - protein, 15 aa, Artificial Sequence
  MIN-17-1 light chain variable framework region 2 (FWR2) amino acid sequence
WNQQKPGQPPRLLIY

SEQ ID NO: 253 - protein, 15 aa, Artificial Sequence
  MIN-17-2 light chain variable framework region 2 (FWR2) amino acid sequence
WYQQKPGKSPQLLIY

SEQ ID NO: 254 - protein, 15 aa, Artificial Sequence
  MIN-29 light chain variable framework region 2 (FWR2) amino acid sequence
WNQQKPGQPPRLLIY

SEQ ID NO: 255 - protein, 15 aa, Artificial Sequence
  MIN-34 light chain variable framework region 2 (FWR2) amino acid sequence
WNQQKPGQPPRLLIY

SEQ ID NO: 256 - skipped
  000

SEQ ID NO: 257 - skipped
  000

SEQ ID NO: 258 - skipped
  000

SEQ ID NO: 259 - skipped
  000

SEQ ID NO: 260 - skipped
  000

SEQ ID NO: 261 - skipped
  000

SEQ ID NO: 262 - skipped
  000

SEQ ID NO: 263 - skipped
  000

SEQ ID NO: 264 - skipped
  000

SEQ ID NO: 265 - skipped
  000

SEQ ID NO: 266 - skipped
  000

SEQ ID NO: 267 - protein, 15 aa, Artificial Sequence
  MIN-45 light chain variable framework region 2 (FWR2) amino acid sequence
WYQQKQGKSPQLLVY

SEQ ID NO: 268 - protein, 7 aa, Artificial Sequence
  MIN-14 light chain variable complementarity determining region 2 (CDR2) amino acid sequence
ATSSLDS

SEQ ID NO: 269 - protein, 7 aa, Artificial Sequence
  MIN-17-1 light chain variable complementarity determining region 2 (CDR2) amino acid sequence
LVSNLES

SEQ ID NO: 270 - protein, 7 aa, Artificial Sequence
  MIN-17-2 light chain variable complementarity determining region 2 (CDR2) amino acid sequence
AATSLAD

SEQ ID NO: 271 - protein, 7 aa, Artificial Sequence
  MIN-29 light chain variable complementarity determining region 2 (CDR2) amino acid sequence
LVSNLES

SEQ ID NO: 272 - protein, 7 aa, Artificial Sequence
  MIN-34 light chain variable complementarity determining region 2 (CDR2) amino acid sequence
LVSNLES

SEQ ID NO: 273 - protein, 7 aa, Artificial Sequence
  MIN-42 light chain variable complementarity determining region 2 (CDR2) amino acid sequence
SASYRYS

SEQ ID NO: 274 - protein, 7 aa, Artificial Sequence
  MIN-45 light chain variable complementarity determining region 2 (CDR2) amino acid sequence
NAKTLAD

SEQ ID NO: 275 - protein, 32 aa, Artificial Sequence
  MIN-14 light chain variable framework region 3 (FWR3) amino acid sequence
GVPKRFSGSRSGSDYSLTISSLESEDFVDYYC

SEQ ID NO: 276 - protein, 32 aa, Artificial Sequence; identical to SEQ ID NO: 139
  MIN-17-1 light chain variable framework region 3 (FWR3) amino acid sequence

SEQ ID NO: 277 - protein, 32 aa, Artificial Sequence
  MIN-17-2 light chain variable framework region 3 (FWR3) amino acid sequence
GVPSRFSGSGSGTKFSFKISSLQAEDFVSYYC

SEQ ID NO: 278 - skipped
  000

SEQ ID NO: 279 - skipped
  000

SEQ ID NO: 280 - skipped
  000

SEQ ID NO: 281 - skipped
  000

SEQ ID NO: 282 - skipped
  000

SEQ ID NO: 283 - skipped
  000

SEQ ID NO: 284 - skipped
  000

SEQ ID NO: 285 - skipped
  000

SEQ ID NO: 286 - skipped
  000

SEQ ID NO: 287 - skipped
  000

SEQ ID NO: 288 - protein, 32 aa, Artificial Sequence; identical to SEQ ID NO: 139
  MIN-29 light chain variable framework region 3 (FWR3) amino acid sequence

SEQ ID NO: 289 - protein, 32 aa, Artificial Sequence; identical to SEQ ID NO: 139
  MIN-34 light chain variable framework region 3 (FWR3) amino acid sequence

SEQ ID NO: 290 - protein, 32 aa, Artificial Sequence
  MIN-42 light chain variable framework region 3 (FWR3) amino acid sequence
GVPDRFTGSGSGTDFTLTISNVQSEDLAEYFC

SEQ ID NO: 291 - protein, 32 aa, Artificial Sequence
  MIN-45 light chain variable framework region 3 (FWR3) amino acid sequence
GVPSRFSGSGSGTQYSLKINSLQPEDFGSYYC

SEQ ID NO: 292 - protein, 30 aa, Artificial Sequence
  MIN-14 heavy chain variable framework region 1 (FWR1) amino acid sequence
QVQLQQPGAELVKPGASVKLSCKASGYTFT

SEQ ID NO: 293 - protein, 30 aa, Artificial Sequence; identical to SEQ ID NO: 292
  MIN-17-1 heavy chain variable framework region 1 (FWR1) amino acid sequence

SEQ ID NO: 294 - protein, 32 aa, Artificial Sequence
  MIN-17-2 heavy chain variable framework region 1 (FWR1) amino acid sequence
QITLKESGPGIVQPSQPFRLTCTFSGFSLSTS

SEQ ID NO: 295 - protein, 59 aa, Artificial Sequence
  MIN-29 heavy chain variable framework region 1 (FWR1) amino acid sequence
  misc_feature (12)..(12): Xaa can be any naturally occurring amino acid
DVKLVESGGDLXKLTEGEDIWEGLTLCRDSDQSPLAPVSKPGRVVRPQRSCTVIQGCVL

SEQ ID NO: 296 - protein, 30 aa, Artificial Sequence
  MIN-34 heavy chain variable framework region 1 (FWR1) amino acid sequence
QVQLKQSGPGLVQPSQSLSITCTVSGFSLT

SEQ ID NO: 297 - skipped
  000

SEQ ID NO: 298 - protein, 30 aa, Artificial Sequence
  MIN-42 heavy chain variable framework region 1 (FWR1) amino acid sequence
EVQLVESGGDLVKPGRSLKLSCAASGFTFS

SEQ ID NO: 299 - protein, 30 aa, Artificial Sequence
  MIN-45 heavy chain variable framework region 1 (FWR1) amino acid sequence
EVQLQQSGPELVKPGASVKISCKASGYSFT

SEQ ID NO: 300 - protein, 5 aa, Artificial Sequence
  MIN-14 heavy chain complementarity determining region 1 (CDR1) amino acid sequence
SYWMH

SEQ ID NO: 301 - protein, 5 aa, Artificial Sequence
  MIN-17-1 heavy chain complementarity determining region 1 (CDR1) amino acid sequence
SYWMH

SEQ ID NO: 302 - protein, 5 aa, Artificial Sequence
  MIN-17-2 heavy chain complementarity determining region 1 (CDR1) amino acid sequence
GIGVT

SEQ ID NO: 303 - protein, 5 aa, Artificial Sequence
  MIN-34 heavy chain complementarity determining region 1 (CDR1) amino acid sequence
SYGVH

SEQ ID NO: 304 - protein, 5 aa, Artificial Sequence
  MIN-42 heavy chain complementarity determining region 1 (CDR1) amino acid sequence
SFGMS

SEQ ID NO: 305 - protein, 5 aa, Artificial Sequence
  MIN-45 heavy chain complementarity determining region 1 (CDR1) amino acid sequence
GYFMS

SEQ ID NO: 306 - protein, 14 aa, Artificial Sequence
  MIN-14 heavy chain variable framework region 2 (FWR2) amino acid sequence
WVKQRPGQGLEWIG

SEQ ID NO: 307 - protein, 14 aa, Artificial Sequence
  MIN-17-1 heavy chain variable framework region 2 (FWR2) amino acid sequence
WVKQRPGQGLEWIG

SEQ ID NO: 308 - protein, 14 aa, Artificial Sequence
  MIN-17-2 heavy chain variable framework region 2 (FWR2) amino acid sequence
WIRQPSGKGLEWLA

SEQ ID NO: 309 - protein, 13 aa, Artificial Sequence
  MIN-29 heavy chain variable framework region 2 (FWR2) amino acid sequence
RLQTAHLQVQGVL

SEQ ID NO: 310 - protein, 14 aa, Artificial Sequence
  MIN-34 heavy chain variable framework region 2 (FWR2) amino acid sequence
WVRQSPGKGLEWLG

SEQ ID NO: 311 - protein, 14 aa, Artificial Sequence
  MIN-42 heavy chain variable framework region 2 (FWR2) amino acid sequence
WVRQTPDKRLEWVA

SEQ ID NO: 312 - protein, 14 aa, Artificial Sequence
  MIN-45 heavy chain variable framework region 2 (FWR1) amino acid sequence
WVMQSHGKSLEWIG

SEQ ID NO: 313 - protein, 17 aa, Artificial Sequence
  MIN-14 heavy chain complementarity determining region 2 (CDR2) amino acid sequence
EINPSNGRTNYNEKFKS

SEQ ID NO: 314 - protein, 17 aa, Artificial Sequence
  MIN-17-1 heavy chain complementarity determining region 2 (CDR2) amino acid sequence
EINPSNGRTNYNEKFKS

SEQ ID NO: 315 - protein, 16 aa, Artificial Sequence
  MIN-17-2 heavy chain complementarity determining region 2 (CDR2) amino acid sequence
TIWWDDDNRYNPSLKS

SEQ ID NO: 316 - protein, 18 aa, Artificial Sequence
  MIN-29 heavy chain complementarity determining region 2 (CDR2) amino acid sequence
GIVSGDGESALHSVWIVG

SEQ ID NO: 317 - protein, 16 aa, Artificial Sequence
  MIN-34 heavy chain complementarity determining region 2 (CDR2) amino acid sequence
VIWGGGSTDYNAAFIS

SEQ ID NO: 318 - protein, 17 aa, Artificial Sequence
  MIN-42 heavy chain complementarity determining region 2 (CDR2) amino acid sequence
TISSGGTYTYYPDSVKG

SEQ ID NO: 319 - protein, 17 aa, Artificial Sequence
  MIN-45 heavy chain complementarity determining region 2 (CDR2) amino acid sequence
RINPYNGDTFYNQKFKG

SEQ ID NO: 320 - protein, 32 aa, Artificial Sequence
  MIN-14 heavy chain variable framework region 3 (FWR3) amino acid sequence
KATLTVDKSSSTAYMQLSSLTSEDSAVYYCAT

SEQ ID NO: 321 - protein, 32 aa, Artificial Sequence; identical to SEQ ID NO: 320
  MIN-17-1 heavy chain variable framework region 3 (FWR3) amino acid sequence

SEQ ID NO: 322 - protein, 32 aa, Artificial Sequence
  MIN-17-2 heavy chain variable framework region 3 (FWR3) amino acid sequence
RLTVSKDTSNNQAFLNIITVETADTAIYYCAQ

SEQ ID NO: 323 - protein, 30 aa, Artificial Sequence
  MIN-29 heavy chain variable framework region 3 (FWR3) amino acid sequence
ATTITINGCDQLQPLLWSLANPRHVIATES

SEQ ID NO: 324 - protein, 32 aa, Artificial Sequence
  MIN-34 heavy chain variable framework region 3 (FWR3) amino acid sequence
RLSISKDNSKSQVFFKMNSLQANDTAIYYCAR

SEQ ID NO: 325 - protein, 32 aa, Artificial Sequence
  MIN-42 heavy chain variable framework region 3 (FWR3) amino acid sequence
RFTISRDNAKNTLYLQMSSLKSEDTAMYYCSR

SEQ ID NO: 326 - protein, 32 aa, Artificial Sequence
  MIN-45 heavy chain variable framework region 3 (FWR3) amino acid sequence
KATLTVDKSSTTAHIELRSLASEDSAVYYCAR

SEQ ID NO: 327 - protein, 465 aa, Artificial Sequence
  MIN-C2 single chain Fab (light chain-linker-heavy chain; VL + CL + linker + VH + CH1) amino acid sequence
DIVITQSTASLGVSLGQRATISCRASKSVSTSGYSYMHWYQQRPGQPPKLLIYLASNLESGVPARFSGSGSGTDFTLNIHPVEEEDAATYYCQHSRELPFTFGGGTKLEIKRADAAPTVSIFPPSSEQLTSGGASVVCFLNNFYPKDINVKWKIDGSERQNGVLNSWTDQDSKDSTYSMSSTLTLTKDEYERHNSYTCEATHKTSTSPIVKSFNRNECSGGGSGGGSEGGGSEGGGSEGGGSEGGGSGGGSGEVQLEESGGGLVKPGGSLKLSCAASGFTFSGYAMSWVRQTPEKRLEWVATISSGGTYIYYPDSVKGRFTISRDNAKNTLYLQMSSLRSEDTAMYYCARLGGDNYYEYFDVWGAGTTVTVSSAKTTPPSVYPLAPGSAAQTNSMVTLGCLVKGYFPEPVTVTWNSGSLSSGVHTFPAVLQSDLYTLSSSVTVPSSTWPSETVTCNVAHPASRTA

SEQ ID NO: 328 - protein, 21 aa, Artificial Sequence
  Ig kappa-chain leader sequence
METDTLLLWVLLLWVPGSTGD

SEQ ID NO: 329 - protein, 10 aa, Artificial Sequence
  Myc tag
EQKLISEEDL

SEQ ID NO: 330 - protein, 5 aa, Artificial Sequence
  VH-CS-CDR1.1: CDR1 Consensus sequence for variable heavy chain for IgG anti-MUC1* antibodies
NYGMN

SEQ ID NO: 331 - protein, 5 aa, Artificial Sequence
  VH-CS-CDR1.2: CDR1 Consensus sequence for variable heavy chain for IgG anti-MUC1* antibodies
GYAMS

SEQ ID NO: 332 - protein, 5 aa, Artificial Sequence
  Xaa at position 1 may be Arg or Gly Xaa at position 3 may be Ala or Gly
  misc_feature (1)..(1): Xaa can be any naturally occurring amino acid
  misc_feature (3)..(3): Xaa can be any naturally occurring amino acid
XYXMS

SEQ ID NO: 333 - protein, 17 aa, Artificial Sequence
  Xaa at position 12 may be Ala or Val Xaa at position 13 may be Gly or Asp
  misc_feature (12)..(13): Xaa can be any naturally occurring amino acid
WINTYTGEPTYXXDFKG

SEQ ID NO: 334 - protein, 17 aa, Artificial Sequence
  VH-CS-CDR2.2: CDR2 Consensus sequence for variable heavy chain for IgG anti-MUC1* antibodies
TISSGGTYIYYPDSVKG

SEQ ID NO: 335 - protein, 9 aa, Artificial Sequence
  Xaa at position 1 may be Ser or Thr        Xaa at position 3 may be Thr or Asp     Xaa at position 4 may be Thr or Ala        Xaa at positions 5-6 may be any naturally-occuring amino acid Xaa at position 7 may be  Tyr or Phe
  misc_feature (1)..(1): Xaa can be any naturally occurring amino acid
  misc_feature (3)..(7): Xaa can be any naturally occurring amino acid
XGXXXXXYA

SEQ ID NO: 336 - protein, 9 aa, Artificial Sequence
  VH-CS-CDR3.2: CDR3 Consensus sequence for variable heavy chain for IgG anti-MUC1* antibodies
TGTTAILNG

SEQ ID NO: 337 - protein, 9 aa, Artificial Sequence
  VH-CS-CDR3.3: CDR3 Consensus sequence for variable heavy chain for IgG anti-MUC1* antibodies
SGDGYWYYA

SEQ ID NO: 338 - protein, 10 aa, Artificial Sequence
  Xaa at positions 5-6 may be any naturally-occurring amino acid Xaa at position 10 may be Gly or Ala
  misc_feature (5)..(6): Xaa can be any naturally occurring amino acid
  misc_feature (10)..(10): Xaa can be any naturally occurring amino acid
DNYGXXYDYX

SEQ ID NO: 339 - protein, 10 aa, Artificial Sequence
  Xaa at position 6 may be Val or IIe Xaa at position 9 may be Met or IIe Xaa at position 10 may be His or Tyr
  misc_feature (6)..(6): Xaa can be any naturally occurring amino acid
  misc_feature (9)..(10): Xaa can be any naturally occurring amino acid
SASSSXSYXX

SEQ ID NO: 340 - protein, 15 aa, Artificial Sequence
  VL-CS-CDR1.2: CDR1 Consensus sequence for variable light chain for IgG anti-MUC1* antibodies
RASKSVSTSGYSYMH

SEQ ID NO: 341 - protein, 7 aa, Artificial Sequence
  Xaa at position 1 may be Ser or Gly
  misc_feature (1)..(1): Xaa can be any naturally occurring amino acid
XTSNLAS

SEQ ID NO: 342 - protein, 7 aa, Artificial Sequence
  VL-CS-CDR2.2: CDR2 Consensus sequence for variable light chain for IgG anti-MUC1* antibodies
LASNLES

SEQ ID NO: 343 - protein, 9 aa, Artificial Sequence
  Xaa at position 5 may be Ser or Asn Xaa at position 8 may be Ser or Phe
  misc_feature (5)..(5): Xaa can be any naturally occurring amino acid
  misc_feature (8)..(8): Xaa can be any naturally occurring amino acid
QQRSXYPXT

SEQ ID NO: 344 - protein, 9 aa, Artificial Sequence
  VL-CS-CDR3.2: CDR3 Consensus sequence for variable light chain for IgG anti-MUC1* antibodies
QHSRELPFT

SEQ ID NO: 345 - protein, 23 aa, Artificial Sequence
  Framework Region 1 Human IgG1 Light Chain Amino Acid SEQ
DIQMTQSPSSLSASVGDRVTITC

SEQ ID NO: 346 - DNA, 75 bp, Artificial Sequence
  Framework Region 1 Human IgG1 Light Chain DNA SEQ
gatatccagatgacccagtccccgagctccctgtccgcctctgtgggcgatagggtcaccatcacctgccgtgcc

SEQ ID NO: 347 - protein, 15 aa, Artificial Sequence
  Framework Region 2 Human IgG1 Light Chain Amino Acid SEQ
WYQQKPGKAPKLLIY

SEQ ID NO: 348 - DNA, 45 bp, Artificial Sequence
  Framework Region 2 Human IgG1 Light Chain DNA SEQ
tggtatcaacagaaaccaggaaaagctccgaaactactgatttac

SEQ ID NO: 349 - protein, 32 aa, Artificial Sequence
  Framework Region 3 Human IgG1 Light Chain Amino Acid SEQ
GVPSRFSGSRSGTDFTLTISSLQPEDFATYYC

SEQ ID NO: 350 - DNA, 93 bp, Artificial Sequence
  Framework Region 3 Human IgG1 Light Chain DNA SEQ
ggagtcccttctcgcttctctggatccagatctgggacggatttcactctgaccatcagcagtctgcagccggaagacttcgcaatctattac

SEQ ID NO: 351 - protein, 10 aa, Artificial Sequence
  Framework Region 4 Human IgG1 Light Chain Amino Acid SEQ
FGQGTKVEIK

SEQ ID NO: 352 - DNA, 30 bp, Artificial Sequence
  Framework Region 4 Human IgG1 Light Chain DNA SEQ
ttcggacagggtaccaaggtggagatcaaa

SEQ ID NO: 353 - protein, 25 aa, Artificial Sequence [sequence omitted]

SEQ ID NO: 354 - DNA, 75 bp, Artificial Sequence
  Framework Region 1  Human IgG1 Heavy Chain DNA SEQ
gaggttcagctggtggagtctggcggtggcctggtgcagccagggggctcactccgtttgtcctgtgcagcttct

SEQ ID NO: 355 - protein, 14 aa, Artificial Sequence
  Framework Region 2  Human IgG1 Heavy Chain Amino Acid SEQ
WVRQAPGKGLEWVA

SEQ ID NO: 356 - DNA, 42 bp, Artificial Sequence
  Framework Region 2  Human IgG1 Heavy Chain DNA SEQ
tgggtgcgtcaggccccgggtaagggcctggaatgggttgca

SEQ ID NO: 357 - protein, 32 aa, Artificial Sequence
  Framework Region 3  Human IgG1 Heavy Chain Amino Acid SEQ
RFTISADTSKNTAYLQMNSLRAEDTAVYYCSR

SEQ ID NO: 358 - DNA, 96 bp, Artificial Sequence
  Framework Region 3  Human IgG1 Heavy Chain DNA SEQ
cgtttcactataagcgcagacacatccaaaaacacagcctacctgcagatgaacagcctgcgtgctgaggacactgccgtctattattgttctaga

SEQ ID NO: 359 - protein, 11 aa, Artificial Sequence
  Framework Region 4  Human IgG1 Heavy Chain Amino Acid SEQ
WGQGTLVTVSS

SEQ ID NO: 360 - DNA, 33 bp, Artificial Sequence
  Framework Region 4  Human IgG1 Heavy DNA SEQ
tggggtcaaggaaccctggtcaccgtctcctcg

SEQ ID NO: 361 - protein, 34 aa, Artificial Sequence
  Linker sequence amino acid
SGGGSGGGSEGGGSEGGGSEGGGSEGGGSGGGSG

SEQ ID NO: 362 - protein, 30 aa, Artificial Sequence
  IGHV3 (name from Igblast): Human IgG antibody framework region sequence with 84.7% homology (249/294) to variable heavy chain region of MIN-C2
EVQLVESGGGLVKPGGSLRLSCAASGFTFS

SEQ ID NO: 363 - protein, 14 aa, Artificial Sequence
  IGHV3 (name from Igblast): Human IgG antibody framework region sequence with 84.7% homology (249/294) to variable heavy chain region of MIN-C2
WVRQAPGKGLEWVS

SEQ ID NO: 364 - protein, 27 aa, Artificial Sequence
  IGHV3 (name from Igblast): Human IgG antibody framework region sequence with 84.7% homology (249/294) to variable heavy chain region of MIN-C2
RFTISRDNAKNSLYLQMNSLRAEDTAV

SEQ ID NO: 365 - protein, 23 aa, Artificial Sequence
  IGkV7 (name from Igblast): Human IgG antibody framework region sequence with 76.4% homology (226/296) to variable light chain region of MIN-C2
DIVLTQSPASLAVSPGQRATITC

SEQ ID NO: 366 - protein, 15 aa, Artificial Sequence
  IGkV7 (name from Igblast): Human IgG antibody framework region sequence with 76.4% homology (226/296) to variable light chain region of MIN-C2
WYQQKPGQPPKLLIY

SEQ ID NO: 367 - protein, 31 aa, Artificial Sequence
  IGkV7 (name from Igblast): Human IgG antibody framework region sequence with 76.4% homology (226/296) to variable light chain region of MIN-C2
GVPARFSGSGSGTDFTLTINPVEANDTANYY

SEQ ID NO: 368 - protein, 30 aa, Artificial Sequence; identical to SEQ ID NO: 362
  IGHV3 (name from Igblast): Human IgG antibody framework region sequence with 84.1% homology (249/296) to variable heavy chain region of MIN-E6

SEQ ID NO: 369 - protein, 14 aa, Artificial Sequence
  IGHV3 (name from Igblast): Human IgG antibody framework region sequence with 84.1% homology (249/296) to variable heavy chain region of MIN-E6
WVRQAPGKGLEWVS

SEQ ID NO: 370 - protein, 32 aa, Artificial Sequence
  IGHV3 (name from Igblast): Human IgG antibody framework region sequence with 84.1% homology (249/296) to variable heavy chain region of MIN-E6
RFTISRDNAKNSLYLQMNSLRAEDTAVYYCAR

SEQ ID NO: 371 - protein, 23 aa, Artificial Sequence
  IGkV3 (name from Igblast): Human IgG antibody framework region sequence with 69.5% homology (187/269) to variable light chain region of MIN-E6
EIVMTQSPATLSVSPGERATLSC

SEQ ID NO: 372 - protein, 15 aa, Artificial Sequence
  IGkV3 (name from Igblast): Human IgG antibody framework region sequence with 69.5% homology (187/269) to variable light chain region of MIN-E6
WFQQRPGTSPKLLIY

SEQ ID NO: 373 - protein, 32 aa, Artificial Sequence
  IGkV3 (name from Igblast): Human IgG antibody framework region sequence with 69.5% homology (187/269) to variable light chain region of MIN-E6
GIPARFSGSGSGTEFTLTISSLQSEDFAVYYC

SEQ ID NO: 374 - protein, 9 aa, Artificial Sequence
  MIN-C2 variable heavy chain region CDR3
LGGDNYYEY